European Patent Application EP 4 501 948 A1, published February 5, 2025. Title: Set of Photoreceptor Proten and Affibody. Applicant: The University of Tokyo. Application JP, filed March 24, 2023. The sequence listing filed with the application follows.

SEQUENCE LISTING (65 sequences)

SEQ ID NO: 1 - protein, 58 aa, Staphylococcus aureus
  source 1..58: note = Affibody
VDNKFNKEKWQAIKEIAVLPNLNQPQHLAFIVSLLDDPSQSANLLAEAKKLNDAQAPK

SEQ ID NO: 2 - protein, 755 aa, Deinococcus radiodurans
MSRDPLPFFPPLYLGGPEITTENCEREPIHIPGSIQPHGALLTADGHSGEVLQMSLNAATFLGQEPTVLRGQTLAALLPEQWPALQAALPPGCPDALQYRATLDWPAAGHLSLTVHRVGELLILEFEPTEAWDSTGPHALRNAMFALESAPNLRALAEVATQTVRELTGFDRVMLYKFAPDATGEVIAEARREGLHAFLGHRFPASDIPAQARALYTRHLLRLTADTRAAAVPLDPVLNPQTNAPTPLGGAVLRATSPMHMQYLRNMGVGSSLSVSVVVGGQLWGLIACHHQTPYVLPPDLRTTLEYLGRLLSLQVQVKEAADVAAFRQSLREHHARVALAAAHSLSPHDTLSDPALDLLGLMRAGGLILRFEGRWQTLGEVPPAPAVDALLAWLETQPGALVQTDALGQLWPAGADLAPSAAGLLAISVGEGWSECLVWLRPELRLEVAWGGATPDQAKDDLGPRHSFDTYLEEKRGYAEPWHPGEIEEAQDLRDTLTGALGERLSVIRDLNRALTQSNAEWRQYGFVISHHMQEPVRLISQFAELLTRQPRAQDGSPDSPQTERITGFLLRETSRLRSLTQDLHTYTALLSAPPPVRRPTPLGRVVDDVLQDLEPRIADTGASIEVAPELPVIAADAGLLRDLLLHLIGNALTFGGPEPRIAVRTERQGAGWSIAVSDQGAGIAPEYQERIFLLFQRLGSLDEALGNGLGLPLCRKIAELHGGTLTVESAPGEGSTFRCWLPDAGPLPGAADA

SEQ ID NO: 3 - DNA, 1647 bp, synthetic construct
  misc_feature 1..1647: note = His6-Avi-DrBphP(PSM)
  source 1..1647: mol_type = other DNA
atgaatcacaaagtgcatcatcatcatcatcatatcgaaggtaggcatatggggttgaatgatattttcgaagcacagaaaattgaatggcatgaggggtccggggggtccggggggtccggggggaagcttatgagccgcgaccccctgccattcttcccccccctgtacctgggaggacccgagattaccaccgaaaactgtgaacgagagcctatccacatccccggaagtattcagcctcatggcgccctgctgactgctgatggccacagtggggaagtgctgcagatgtcactgaacgccgctaccttcctggggcaggagcctactgtgctgaggggacagaccctggcagcactgctgcctgaacagtggccagcactgcaggctgcactgccacctggctgccccgatgccctgcagtacagggctactctggactggcctgcagctggacacctgagcctgaccgtccatcgcgtgggggaactgctgatcctggagttcgaaccaacagaggcttgggatagcactggcccccacgcactgcggaacgctatgtttgcactggagtccgcccccaatctgagagcactggccgaagtcgccactcagaccgtgcgggagctgacagggttcgatagagtcatgctgtacaagtttgcccctgacgctactggagaagtgatcgctgaagcacggagagaggggctgcacgctttcctgggacatcgatttccagcctccgacattccagcacaggctcgggcactgtataccaggcacctgctgcgactgacagcagatactcgcgcagcagctgtcccactggaccccgtgctgaaccctcagaccaatgcaccaacacctctgggaggagcagtgctgagagcaacctctccaatgcatatgcagtatctgaggaatatgggagtcggcagctccctgtctgtgagtgtggtcgtgggaggacagctgtggggactgattgcctgccaccatcagacaccctacgtgctgccacccgatctgaggaccacactggagtatctggggcgcctgctgtctctgcaggtccaggtgaaagaagcagccgacgtcgctgcattccgacagagtctgcgagagcaccatgcacgggtggccctggccgctgcacactcactgagccctcatgacacactgagcgatccagctctggacctgctgggactgatgagagcaggaggactgatcctgagatttgaaggcaggtggcagactctgggagaggtccctccagcaccagctgtggacgctctgctggcatggctggagacccagccaggagctctggtgcagacagatgcactgggacagctgtggccagcaggagcagacctggctccttcagcagctggactgctggccatttccgtcggagaaggatggtctgagtgtctggtgtggctgcgcccagaactgcgactggaggtggcttggggaggagcaacccctgatcaggcaaaggacgatctgggaccacgccacagctttgacacatacctggaggaaaaacgaggctatgccgagccctggcacccaggggaaattgaggaggcacaggatctgagagacacactgacaggggcactgctcgagtaa

SEQ ID NO: 4 - DNA, 2400 bp, synthetic construct
  misc_feature 1..2400: note = His6-Avi-DrBphP
  source 1..2400: mol_type = other DNA
atgaatcacaaagtgcatcatcatcatcatcatatcgaaggtaggcatatggggttgaatgatattttcgaagcacagaaaattgaatggcatgaggggtccggggggtccggggggtccggggggaagcttatgagccgcgaccccctgccattcttcccccccctgtacctgggaggacccgagattaccaccgaaaactgtgaacgagagcctatccacatccccggaagtattcagcctcatggcgccctgctgactgctgatggccacagtggggaagtgctgcagatgtcactgaacgccgctaccttcctggggcaggagcctactgtgctgaggggacagaccctggcagcactgctgcctgaacagtggccagcactgcaggctgcactgccacctggctgccccgatgccctgcagtacagggctactctggactggcctgcagctggacacctgagcctgaccgtccatcgcgtgggggaactgctgatcctggagttcgaaccaacagaggcttgggatagcactggcccccacgcactgcggaacgctatgtttgcactggagtccgcccccaatctgagagcactggccgaagtcgccactcagaccgtgcgggagctgacagggttcgatagagtcatgctgtacaagtttgcccctgacgctactggagaagtgatcgctgaagcacggagagaggggctgcacgctttcctgggacatcgatttccagcctccgacattccagcacaggctcgggcactgtataccaggcacctgctgcgactgacagcagatactcgcgcagcagctgtcccactggaccccgtgctgaaccctcagaccaatgcaccaacacctctgggaggagcagtgctgagagcaacctctccaatgcatatgcagtatctgaggaatatgggagtcggcagctccctgtctgtgagtgtggtcgtgggaggacagctgtggggactgattgcctgccaccatcagacaccctacgtgctgccacccgatctgaggaccacactggagtatctggggcgcctgctgtctctgcaggtccaggtgaaagaagcagccgacgtcgctgcattccgacagagtctgcgagagcaccatgcacgggtggccctggccgctgcacactcactgagccctcatgacacactgagcgatccagctctggacctgctgggactgatgagagcaggaggactgatcctgagatttgaaggcaggtggcagactctgggagaggtccctccagcaccagctgtggacgctctgctggcatggctggagacccagccaggagctctggtgcagacagatgcactgggacagctgtggccagcaggagcagacctggctccttcagcagctggactgctggccatttccgtcggagaaggatggtctgagtgtctggtgtggctgcgcccagaactgcgactggaggtggcttggggaggagcaacccctgatcaggcaaaggacgatctgggaccacgccacagctttgacacatacctggaggaaaaacgaggctatgccgagccctggcacccaggggaaattgaggaggcacaggatctgagagacacactgacaggggcactgggggagagactgtccgtgattcgcgatctcaaccgggctctgacccagtccaatgccgagtggcgtcagtatggcttcgtcatcagtcaccacatgcaggaacccgtcagactgatctcccagtttgccgagcttctgactcgccaacccagagcccaggatggcagcccggactctccccagacagagcgtatcaccggctttctgctcagggaaacctcacgactccgctctctgacccaggacttgcacacgtacactgcgctgctgtcagcacctcctccagttaggaggccaacaccacttgggcgagttgtggacgatgtgctgcaggacctcgaaccacggattgccgatacaggggcctccatagaggtagctcccgaactgcccgtcattgccgctgatgctggcctcttgcgcgaccttctgctgcatctgattggtaacgccttgaccttcggaggaccagagcctcggattgctgtgagaaccgaacggcaaggtgccggctggagcatcgctgtgagcgatcagggtgcggggatagcgccggagtatcaggagaggatcttcttgctcttccagagactcggctctctggacgaggcactgggcaatggacttgggcttcccctgtgtcggaagatcgccgaactgcatggtggcacactgactgtggagagtgcacctggcgaaggaagcacgtttaggtgctggctgcctgatgccggaccactgcctggagcagcagacgcttaa

SEQ ID NO: 5 - DNA, 2190 bp, synthetic construct
  misc_feature 1..2190: note = tetR-DrBphP(PSM)
  source 1..2190: mol_type = other DNA
atgggctccagattagataaaagtaaagtgattaacagcgcattagagctgcttaatgaggtcggaatcgaaggtttaacaacccgtaaactcgcccagaagctaggtgtagagcagcctacattgtattggcatgtaaaaaataagcgggctttgctcgacgccttagccattgagatgttagataggcaccatactcacttttgccctttagaaggggaaagctggcaagattttttacgtaataacgctaaaagttttagatgtgctttactaagtcatcgcgatggagcaaaagtacatttaggtacacggcctacagaaaaacagtatgaaactctcgaaaatcaattagcctttttatgccaacaaggtttttcactagagaatgcattatatgcactcagcgctgtggggcattttactttaggttgcgtattggaagatcaagagcatcaagtcgctaaagaagaaagggaaacacctactactgatagtatgccgccattattacgacaagctatcgaattatttgatcaccaaggtgcagagccagccttcttattcggccttgaattgatcatatgcggattagaaaaacaacttaaatgtgaaagtgggtccgcgtacagccgcgcgctcgatagtgctggtagtgctggtagtgctagcgccaccagccgcgaccccctgccattcttcccccccctgtacctgggaggacccgagattaccaccgaaaactgtgaacgagagcctatccacatccccggaagtattcagcctcatggcgccctgctgactgctgatggccacagtggggaagtgctgcagatgtcactgaacgccgctaccttcctggggcaggagcctactgtgctgaggggacagaccctggcagcactgctgcctgaacagtggccagcactgcaggctgcactgccacctggctgccccgatgccctgcagtacagggctactctggactggcctgcagctggacacctgagcctgaccgtccatcgcgtgggggaactgctgatcctggagttcgaaccaacagaggcttgggatagcactggcccccacgcactgcggaacgctatgtttgcactggagtccgcccccaatctgagagcactggccgaagtcgccactcagaccgtgcgggagctgacagggttcgatagagtcatgctgtacaagtttgcccctgacgctactggagaagtgatcgctgaagcacggagagaggggctgcacgctttcctgggacatcgatttccagcctccgacattccagcacaggctcgggcactgtataccaggcacctgctgcgactgacagcagatactcgcgcagcagctgtcccactggaccccgtgctgaaccctcagaccaatgcaccaacacctctgggaggagcagtgctgagagcaacctctccaatgcatatgcagtatctgaggaatatgggagtcggcagctccctgtctgtgagtgtggtcgtgggaggacagctgtggggactgattgcctgccaccatcagacaccctacgtgctgccacccgatctgaggaccacactggagtatctggggcgcctgctgtctctgcaggtccaggtgaaagaagcagccgacgtcgctgcattccgacagagtctgcgagagcaccatgcacgggtggccctggccgctgcacactcactgagccctcatgacacactgagcgatccagctctggacctgctgggactgatgagagcaggaggactgatcctgagatttgaaggcaggtggcagactctgggagaggtccctccagcaccagctgtggacgctctgctggcatggctggagacccagccaggagctctggtgcagacagatgcactgggacagctgtggccagcaggagcagacctggctccttcagcagctggactgctggccatttccgtcggagaaggatggtctgagtgtctggtgtggctgcgcccagaactgcgactggaggtggcttggggaggagcaacccctgatcaggcaaaggacgatctgggaccacgccacagctttgacacatacctggaggaaaaacgaggctatgccgagccctggcacccaggggaaattgaggaggcacaggatctgagagacacactgacaggggcactgggtacctag

SEQ ID NO: 6 - protein, 981 aa, synthetic construct
  REGION 1..981: note = tetR-DrBphP
MGSRLDKSKVINSALELLNEVGIEGLTTRKLAQKLGVEQPTLYWHVKNKRALLDALAIEMLDRHHTHFCPLEGESWQDFLRNNAKSFRCALLSHRDGAKVHLGTRPTEKQYETLENQLAFLCQQGFSLENALYALSAVGHFTLGCVLEDQEHQVAKEERETPTTDSMPPLLRQAIELFDHQGAEPAFLFGLELIICGLEKQLKCESGSAYSRALDSAGSAGSASATMSRDPLPFFPPLYLGGPEITTENCEREPIHIPGSIQPHGALLTADGHSGEVLQMSLNAATFLGQEPTVLRGQTLAALLPEQWPALQAALPPGCPDALQYRATLDWPAAGHLSLTVHRVGELLILEFEPTEAWDSTGPHALRNAMFALESAPNLRALAEVATQTVRELTGFDRVMLYKFAPDATGEVIAEARREGLHAFLGHRFPASDIPAQARALYTRHLLRLTADTRAAAVPLDPVLNPQTNAPTPLGGAVLRATSPMHMQYLRNMGVGSSLSVSVVVGGQLWGLIACHHQTPYVLPPDLRTTLEYLGRLLSLQVQVKEAADVAAFRQSLREHHARVALAAAHSLSPHDTLSDPALDLLGLMRAGGLILRFEGRWQTLGEVPPAPAVDALLAWLETQPGALVQTDALGQLWPAGADLAPSAAGLLAISVGEGWSECLVWLRPELRLEVAWGGATPDQAKDDLGPRHSFDTYLEEKRGYAEPWHPGEIEEAQDLRDTLTGALGERLSVIRDLNRALTQSNAEWRQYGFVISHHMQEPVRLISQFAELLTRQPRAQDGSPDSPQTERITGFLLRETSRLRSLTQDLHTYTALLSAPPPVRRPTPLGRVVDDVLQDLEPRIADTGASIEVAPELPVIAADAGLLRDLLLHLIGNALTFGGPEPRIAVRTERQGAGWSIAVSDQGAGIAPEYQERIFLLFQRLGSLDEALGNGLGLPLCRKIAELHGGTLTVESAPGEGSTFRCWLPDAGPLPGAADA

SEQ ID NO: 7 - DNA, 2958 bp, synthetic construct
  misc_feature 1..2958: note = tetR-DrBphP
  source 1..2958: mol_type = other DNA
atgggctccagattagataaaagtaaagtgattaacagcgcattagagctgcttaatgaggtcggaatcgaaggtttaacaacccgtaaactcgcccagaagctaggtgtagagcagcctacattgtattggcatgtaaaaaataagcgggctttgctcgacgccttagccattgagatgttagataggcaccatactcacttttgccctttagaaggggaaagctggcaagattttttacgtaataacgctaaaagttttagatgtgctttactaagtcatcgcgatggagcaaaagtacatttaggtacacggcctacagaaaaacagtatgaaactctcgaaaatcaattagcctttttatgccaacaaggtttttcactagagaatgcattatatgcactcagcgctgtggggcattttactttaggttgcgtattggaagatcaagagcatcaagtcgctaaagaagaaagggaaacacctactactgatagtatgccgccattattacgacaagctatcgaattatttgatcaccaaggtgcagagccagccttcttattcggccttgaattgatcatatgcggattagaaaaacaacttaaatgtgaaagtgggtccgcgtacagccgcgcgctcgatagtgctggtagtgctggtagtgctagcgccaccatgagccgcgaccccctgccattcttcccccccctgtacctgggaggacccgagattaccaccgaaaactgtgaacgagagcctatccacatccccggaagtattcagcctcatggcgccctgctgactgctgatggccacagtggggaagtgctgcagatgtcactgaacgccgctaccttcctggggcaggagcctactgtgctgaggggacagaccctggcagcactgctgcctgaacagtggccagcactgcaggctgcactgccacctggctgccccgatgccctgcagtacagggctactctggactggcctgcagctggacacctgagcctgaccgtccatcgcgtgggggaactgctgatcctggagttcgaaccaacagaggcttgggatagcactggcccccacgcactgcggaacgctatgtttgcactggagtccgcccccaatctgagagcactggccgaagtcgccactcagaccgtgcgggagctgacagggttcgatagagtcatgctgtacaagtttgcccctgacgctactggagaagtgatcgctgaagcacggagagaggggctgcacgctttcctgggacatcgatttccagcctccgacattccagcacaggctcgggcactgtataccaggcacctgctgcgactgacagcagatactcgcgcagcagctgtcccactggaccccgtgctgaaccctcagaccaatgcaccaacacctctgggaggagcagtgctgagagcaacctctccaatgcatatgcagtatctgaggaatatgggagtcggcagctccctgtctgtgagtgtggtcgtgggaggacagctgtggggactgattgcctgccaccatcagacaccctacgtgctgccacccgatctgaggaccacactggagtatctggggcgcctgctgtctctgcaggtccaggtgaaagaagcagccgacgtcgctgcattccgacagagtctgcgagagcaccatgcacgggtggccctggccgctgcacactcactgagccctcatgacacactgagcgatccagctctggacctgctgggactgatgagagcaggaggactgatcctgagatttgaaggcaggtggcagactctgggagaggtccctccagcaccagctgtggacgctctgctggcatggctggagacccagccaggagctctggtgcagacagatgcactgggacagctgtggccagcaggagcagacctggctccttcagcagctggactgctggccatttccgtcggagaaggatggtctgagtgtctggtgtggctgcgcccagaactgcgactggaggtggcttggggaggagcaacccctgatcaggcaaaggacgatctgggaccacgccacagctttgacacatacctggaggaaaaacgaggctatgccgagccctggcacccaggggaaattgaggaggcacaggatctgagagacacactgacaggggcactgggggagagactgtccgtgattcgcgatctcaaccgggctctgacccagtccaatgccgagtggcgtcagtatggcttcgtcatcagtcaccacatgcaggaacccgtcagactgatctcccagtttgccgagcttctgactcgccaacccagagcccaggatggcagcccggactctccccagacagagcgtatcaccggctttctgctcagggaaacctcacgactccgctctctgacccaggacttgcacacgtacactgcgctgctgtcagcacctcctccagttaggaggccaacaccacttgggcgagttgtggacgatgtgctgcaggacctcgaaccacggattgccgatacaggggcctccatagaggtagctcccgaactgcccgtcattgccgctgatgctggcctcttgcgcgaccttctgctgcatctgattggtaacgccttgaccttcggaggaccagagcctcggattgctgtgagaaccgaacggcaaggtgccggctggagcatcgctgtgagcgatcagggtgcggggatagcgccggagtatcaggagaggatcttcttgctcttccagagactcggctctctggacgaggcactgggcaatggacttgggcttcccctgtgtcggaagatcgccgaactgcatggtggcacactgactgtggagagtgcacctggcgaaggaagcacgtttaggtgctggctgcctgatgccggaccactgcctggagcagcagacgctgaattcggtacctag

SEQ ID NO: 8 - DNA, 846 bp, synthetic construct
  misc_feature 1..846: note = MS2-Aff6_V18F N-V5-His
  source 1..846: mol_type = other DNA
atggccagccccaagaagaagcgcaaggtggaagctagcgcttccccgaagaaaaagcggaaagtcgaggcctccgcatctccaaaaaaaaaaagcaaggttgaagcatctggatccgggggcggaatggcttctaactttactcagttcgttctcgtcgacaatggcggaactggcgacgtgactgtcgccccaagcaacttcgctaacgggatcgctgaatggatcagctctaactcgcgttcacaggcttacaaagtaacctgtagcgttcgtcagagctctgcgcagaatcgcaaatacaccatcaaagtcgaggtgcctaaaggcgcctggcgttcgtacttaaatatggaactaaccattccaattttcgccacgaattccgactgcgagcttattgttaaggcaatgcaaggtctcctaaaagatggaaacccgattccctcagcaatcgcagcaaactccggcatctacgcgggtaccggaggaagtggcagctctggcggcagtggagggtctggtggcagcggaatgaagtttaacaaggagaagtggcaggctattaaggagattgccttcctgcctaacctgaaccagccccagcacctggcttttattgtgtctctgctggacgacccttctcagtctgctaacctgctggctgaggctaagaagctgaacgacgctcaggctcctaaggggggttctggggggagcggcgggggatctggaagtggcagcggaggcctcgagtctagagggcccttcgaaggtaagcctatccctaaccctctcctcggtctcgattctacgcgtaccggtcatcatcaccatcaccattga

SEQ ID NO: 9 - DNA, 2841 bp, synthetic construct
  misc_feature 1..2841: note = 3xNLS-DrBphP-MS2
  source 1..2841: mol_type = other DNA
atggccagccccaagaagaagcgcaaggtggaagctagcgcttccccgaagaaaaagcggaaagtcgaggcctccgcatctccaaaaaaaaaaagcaaggttgaagcatctggatccggaggaagtggcagctctggcggcagtggagggtctggtggcagcggaatgagccgcgaccccctgccattcttcccccccctgtacctgggaggacccgagattaccaccgaaaactgtgaacgagagcctatccacatccccggaagtattcagcctcatggcgccctgctgactgctgatggccacagtggggaagtgctgcagatgtcactgaacgccgctaccttcctggggcaggagcctactgtgctgaggggacagaccctggcagcactgctgcctgaacagtggccagcactgcaggctgcactgccacctggctgccccgatgccctgcagtacagggctactctggactggcctgcagctggacacctgagcctgaccgtccatcgcgtgggggaactgctgatcctggagttcgaaccaacagaggcttgggatagcactggcccccacgcactgcggaacgctatgtttgcactggagtccgcccccaatctgagagcactggccgaagtcgccactcagaccgtgcgggagctgacagggttcgatagagtcatgctgtacaagtttgcccctgacgctactggagaagtgatcgctgaagcacggagagaggggctgcacgctttcctgggacatcgatttccagcctccgacattccagcacaggctcgggcactgtataccaggcacctgctgcgactgacagcagatactcgcgcagcagctgtcccactggaccccgtgctgaaccctcagaccaatgcaccaacacctctgggaggagcagtgctgagagcaacctctccaatgcatatgcagtatctgaggaatatgggagtcggcagctccctgtctgtgagtgtggtcgtgggaggacagctgtggggactgattgcctgccaccatcagacaccctacgtgctgccacccgatctgaggaccacactggagtatctggggcgcctgctgtctctgcaggtccaggtgaaagaagcagccgacgtcgctgcattccgacagagtctgcgagagcaccatgcacgggtggccctggccgctgcacactcactgagccctcatgacacactgagcgatccagctctggacctgctgggactgatgagagcaggaggactgatcctgagatttgaaggcaggtggcagactctgggagaggtccctccagcaccagctgtggacgctctgctggcatggctggagacccagccaggagctctggtgcagacagatgcactgggacagctgtggccagcaggagcagacctggctccttcagcagctggactgctggccatttccgtcggagaaggatggtctgagtgtctggtgtggctgcgcccagaactgcgactggaggtggcttggggaggagcaacccctgatcaggcaaaggacgatctgggaccacgccacagctttgacacatacctggaggaaaaacgaggctatgccgagccctggcacccaggggaaattgaggaggcacaggatctgagagacacactgacaggggcactgggggagagactgtccgtgattcgcgatctcaaccgggctctgacccagtccaatgccgagtggcgtcagtatggcttcgtcatcagtcaccacatgcaggaacccgtcagactgatctcccagtttgccgagcttctgactcgccaacccagagcccaggatggcagcccggactctccccagacagagcgtatcaccggctttctgctcagggaaacctcacgactccgctctctgacccaggacttgcacacgtacactgcgctgctgtcagcacctcctccagttaggaggccaacaccacttgggcgagttgtggacgatgtgctgcaggacctcgaaccacggattgccgatacaggggcctccatagaggtagctcccgaactgcccgtcattgccgctgatgctggcctcttgcgcgaccttctgctgcatctgattggtaacgccttgaccttcggaggaccagagcctcggattgctgtgagaaccgaacggcaaggtgccggctggagcatcgctgtgagcgatcagggtgcggggatagcgccggagtatcaggagaggatcttcttgctcttccagagactcggctctctggacgaggcactgggcaatggacttgggcttcccctgtgtcggaagatcgccgaactgcatggtggcacactgactgtggagagtgcacctggcgaaggaagcacgtttaggtgctggctgcctgatgccggaccactgcctggagcagcagacgctgggggttctggggggagcggcgggggatctggaagtggcagcggaggcggtaccatggcttctaactttactcagttcgttctcgtcgacaatggcggaactggcgacgtgactgtcgccccaagcaacttcgctaacgggatcgctgaatggatcagctctaactcgcgttcacaggcttacaaagtaacctgtagcgttcgtcagagctctgcgcagaatcgcaaatacaccatcaaagtcgaggtgcctaaaggcgcctggcgttcgtacttaaatatggaactaaccattccaattttcgccacgaattccgactgcgagcttattgttaaggcaatgcaaggtctcctaaaagatggaaacccgattccctcagcaatcgcagcaaactccggcatctacgcgtaa

SEQ ID NO: 10 - DNA, 3399 bp, synthetic construct
  misc_feature 1..3399: note = 3xNLS-p65-HSF1-DrBphP
  source 1..3399: mol_type = other DNA
atggccagccccaagaagaagcgcaaggtggaagctagcgcttccccgaagaaaaagcggaaagtcgaggcctccgcatctccgaaaaaaaaaagcaaggttgaagcatctggatccggtaccggggggagcggcgggccttcagggcagatcagcaaccaggccctggctctggcccctagctccgctccagtgctggcccagactatggtgccctctagtgctatggtgcctctggcccagccacctgctccagcccctgtgctgaccccaggaccaccccagtcactgagcgctccagtgcccaagtctacacaggccggcgaggggactctgagtgaagctctgctgcacctgcagttcgacgctgatgaggacctgggagctctgctggggaacagcaccgatcccggagtgttcacagatctggcctccgtggacaactctgagtttcagcagctgctgaatcagggcgtgtccatgtctcatagtacagccgaaccaatgctgatggagtaccccgaagccattacccggctggtgaccggcagccagcggccccccgaccccgctccaactcccctgggaaccagcggcctgcctaatgggctgtccggagatgaagacttctcaagcatcgctgatatggactttagtgccctgctgtcacagatttcctctagtgggcagggaggaggtggaagcggcttcagcgtggacaccagtgccctgctggacctgttcagcccctcggtgaccgtgcccgacatgagcctgcctgaccttgacagcagcctggccagtatccaagagctcctgtctccccaggagccccccaggcctcccgaggcagagaacagcagcccggattcagggaagcagctggtgcactacacagcgcagccgctgttcctgctggaccccggctccgtggacaccgggagcaacgacctgccggtgctgtttgagctgggagagggctcctacttctccgaaggggacggcttcgccgaggaccccaccatctccctgctgacaggctcggagcctcccaaagccaaggaccccactgtctccctcgagggaggaagtggcagctctggcggcagtggagggtctggtggcagcggaatgagccgcgaccccctgccattcttcccccccctgtacctgggaggacccgagattaccaccgaaaactgtgaacgagagcctatccacatccccggaagtattcagcctcatggcgccctgctgactgctgatggccacagtggggaagtgctgcagatgtcactgaacgccgctaccttcctggggcaggagcctactgtgctgaggggacagaccctggcagcactgctgcctgaacagtggccagcactgcaggctgcactgccacctggctgccccgatgccctgcagtacagggctactctggactggcctgcagctggacacctgagcctgaccgtccatcgcgtgggggaactgctgatcctggagttcgaaccaacagaggcttgggatagcactggcccccacgcactgcggaacgctatgtttgcactggagtccgcccccaatctgagagcactggccgaagtcgccactcagaccgtgcgggagctgacagggttcgatagagtcatgctgtacaagtttgcccctgacgctactggagaagtgatcgctgaagcacggagagaggggctgcacgctttcctgggacatcgatttccagcctccgacattccagcacaggctcgggcactgtataccaggcacctgctgcgactgacagcagatactcgcgcagcagctgtcccactggaccccgtgctgaaccctcagaccaatgcaccaacacctctgggaggagcagtgctgagagcaacctctccaatgcatatgcagtatctgaggaatatgggagtcggcagctccctgtctgtgagtgtggtcgtgggaggacagctgtggggactgattgcctgccaccatcagacaccctacgtgctgccacccgatctgaggaccacactggagtatctggggcgcctgctgtctctgcaggtccaggtgaaagaagcagccgacgtcgctgcattccgacagagtctgcgagagcaccatgcacgggtggccctggccgctgcacactcactgagccctcatgacacactgagcgatccagctctggacctgctgggactgatgagagcaggaggactgatcctgagatttgaaggcaggtggcagactctgggagaggtccctccagcaccagctgtggacgctctgctggcatggctggagacccagccaggagctctggtgcagacagatgcactgggacagctgtggccagcaggagcagacctggctccttcagcagctggactgctggccatttccgtcggagaaggatggtctgagtgtctggtgtggctgcgcccagaactgcgactggaggtggcttggggaggagcaacccctgatcaggcaaaggacgatctgggaccacgccacagctttgacacatacctggaggaaaaacgaggctatgccgagccctggcacccaggggaaattgaggaggcacaggatctgagagacacactgacaggggcactgggggagagactgtccgtgattcgcgatctcaaccgggctctgacccagtccaatgccgagtggcgtcagtatggcttcgtcatcagtcaccacatgcaggaacccgtcagactgatctcccagtttgccgagcttctgactcgccaacccagagcccaggatggcagcccggactctccccagacagagcgtatcaccggctttctgctcagggaaacctcacgactccgctctctgacccaggacttgcacacgtacactgcgctgctgtcagcacctcctccagttaggaggccaacaccacttgggcgagttgtggacgatgtgctgcaggacctcgaaccacggattgccgatacaggggcctccatagaggtagctcccgaactgcccgtcattgccgctgatgctggcctcttgcgcgaccttctgctgcatctgattggtaacgccttgaccttcggaggaccagagcctcggattgctgtgagaaccgaacggcaaggtgccggctggagcatcgctgtgagcgatcagggtgcggggatagcgccggagtatcaggagaggatcttcttgctcttccagagactcggctctctggacgaggcactgggcaatggacttgggcttcccctgtgtcggaagatcgccgaactgcatggtggcacactgactgtggagagtgcacctggcgaaggaagcacgtttaggtgctggctgcctgatgccggaccactgcctggagcagcagacgcttaa

SEQ ID NO: 11 - DNA, 3432 bp, synthetic construct
  misc_feature 1..3432: note = 3xNLS-DrBphP-p65-HSF1
  source 1..3432: mol_type = other DNA
atggccagccccaagaagaagcgcaaggtggaagctagcgcttccccgaagaaaaagcggaaagtcgaggcctccgcatctccgaaaaaaaaaagcaaggttgaagcatctggatccggtaccggaggaagtggcagctctggcggcagtggagggtctggtggcagcggaatgagccgcgaccccctgccattcttcccccccctgtacctgggaggacccgagattaccaccgaaaactgtgaacgagagcctatccacatccccggaagtattcagcctcatggcgccctgctgactgctgatggccacagtggggaagtgctgcagatgtcactgaacgccgctaccttcctggggcaggagcctactgtgctgaggggacagaccctggcagcactgctgcctgaacagtggccagcactgcaggctgcactgccacctggctgccccgatgccctgcagtacagggctactctggactggcctgcagctggacacctgagcctgaccgtccatcgcgtgggggaactgctgatcctggagttcgaaccaacagaggcttgggatagcactggcccccacgcactgcggaacgctatgtttgcactggagtccgcccccaatctgagagcactggccgaagtcgccactcagaccgtgcgggagctgacagggttcgatagagtcatgctgtacaagtttgcccctgacgctactggagaagtgatcgctgaagcacggagagaggggctgcacgctttcctgggacatcgatttccagcctccgacattccagcacaggctcgggcactgtataccaggcacctgctgcgactgacagcagatactcgcgcagcagctgtcccactggaccccgtgctgaaccctcagaccaatgcaccaacacctctgggaggagcagtgctgagagcaacctctccaatgcatatgcagtatctgaggaatatgggagtcggcagctccctgtctgtgagtgtggtcgtgggaggacagctgtggggactgattgcctgccaccatcagacaccctacgtgctgccacccgatctgaggaccacactggagtatctggggcgcctgctgtctctgcaggtccaggtgaaagaagcagccgacgtcgctgcattccgacagagtctgcgagagcaccatgcacgggtggccctggccgctgcacactcactgagccctcatgacacactgagcgatccagctctggacctgctgggactgatgagagcaggaggactgatcctgagatttgaaggcaggtggcagactctgggagaggtccctccagcaccagctgtggacgctctgctggcatggctggagacccagccaggagctctggtgcagacagatgcactgggacagctgtggccagcaggagcagacctggctccttcagcagctggactgctggccatttccgtcggagaaggatggtctgagtgtctggtgtggctgcgcccagaactgcgactggaggtggcttggggaggagcaacccctgatcaggcaaaggacgatctgggaccacgccacagctttgacacatacctggaggaaaaacgaggctatgccgagccctggcacccaggggaaattgaggaggcacaggatctgagagacacactgacaggggcactgggggagagactgtccgtgattcgcgatctcaaccgggctctgacccagtccaatgccgagtggcgtcagtatggcttcgtcatcagtcaccacatgcaggaacccgtcagactgatctcccagtttgccgagcttctgactcgccaacccagagcccaggatggcagcccggactctccccagacagagcgtatcaccggctttctgctcagggaaacctcacgactccgctctctgacccaggacttgcacacgtacactgcgctgctgtcagcacctcctccagttaggaggccaacaccacttgggcgagttgtggacgatgtgctgcaggacctcgaaccacggattgccgatacaggggcctccatagaggtagctcccgaactgcccgtcattgccgctgatgctggcctcttgcgcgaccttctgctgcatctgattggtaacgccttgaccttcggaggaccagagcctcggattgctgtgagaaccgaacggcaaggtgccggctggagcatcgctgtgagcgatcagggtgcggggatagcgccggagtatcaggagaggatcttcttgctcttccagagactcggctctctggacgaggcactgggcaatggacttgggcttcccctgtgtcggaagatcgccgaactgcatggtggcacactgactgtggagagtgcacctggcgaaggaagcacgtttaggtgctggctgcctgatgccggaccactgcctggagcagcagacgctgggggttctggggggagcggcgggggatctggaagtggcagcggaggcctcgagccttcagggcagatcagcaaccaggccctggctctggcccctagctccgctccagtgctggcccagactatggtgccctctagtgctatggtgcctctggcccagccacctgctccagcccctgtgctgaccccaggaccaccccagtcactgagcgctccagtgcccaagtctacacaggccggcgaggggactctgagtgaagctctgctgcacctgcagttcgacgctgatgaggacctgggagctctgctggggaacagcaccgatcccggagtgttcacagatctggcctccgtggacaactctgagtttcagcagctgctgaatcagggcgtgtccatgtctcatagtacagccgaaccaatgctgatggagtaccccgaagccattacccggctggtgaccggcagccagcggccccccgaccccgctccaactcccctgggaaccagcggcctgcctaatgggctgtccggagatgaagacttctcaagcatcgctgatatggactttagtgccctgctgtcacagatttcctctagtgggcagggaggaggtggaagcggcttcagcgtggacaccagtgccctgctggacctgttcagcccctcggtgaccgtgcccgacatgagcctgcctgaccttgacagcagcctggccagtatccaagagctcctgtctccccaggagccccccaggcctcccgaggcagagaacagcagcccggattcagggaagcagctggtgcactacacagcgcagccgctgttcctgctggaccccggctccgtggacaccgggagcaacgacctgccggtgctgtttgagctgggagagggctcctacttctccgaaggggacggcttcgccgaggaccccaccatctccctgctgacaggctcggagcctcccaaagccaaggaccccactgtctcctaa

SEQ ID NO: 12 - DNA, 2472 bp, synthetic construct
  misc_feature 1..2472: note = NLS-CreN59-DrBphP
  source 1..2472: mol_type = other DNA
atggtgcccaagaagaagaggaaagtcggcggaatgacctctgatgaagtcaggaagaacctgatggacatgttcagggacaggcaggccttctctgaacacacctggaagatgctcctgtctgtgtgcagatcctgggctgcctggtgcaagctgaacggtaccgccagcccctctaaccctggagcctccaacggcagcctcgagagccgcgaccccctgccattcttcccccccctgtacctgggaggacccgagattaccaccgaaaactgtgaacgagagcctatccacatccccggaagtattcagcctcatggcgccctgctgactgctgatggccacagtggggaagtgctgcagatgtcactgaacgccgctaccttcctggggcaggagcctactgtgctgaggggacagaccctggcagcactgctgcctgaacagtggccagcactgcaggctgcactgccacctggctgccccgatgccctgcagtacagggctactctggactggcctgcagctggacacctgagcctgaccgtccatcgcgtgggggaactgctgatcctggagttcgaaccaacagaggcttgggatagcactggcccccacgcactgcggaacgctatgtttgcactggagtccgcccccaatctgagagcactggccgaagtcgccactcagaccgtgcgggagctgacagggttcgatagagtcatgctgtacaagtttgcccctgacgctactggagaagtgatcgctgaagcacggagagaggggctgcacgctttcctgggacatcgatttccagcctccgacattccagcacaggctcgggcactgtataccaggcacctgctgcgactgacagcagatactcgcgcagcagctgtcccactggaccccgtgctgaaccctcagaccaatgcaccaacacctctgggaggagcagtgctgagagcaacctctccaatgcatatgcagtatctgaggaatatgggagtcggcagctccctgtctgtgagtgtggtcgtgggaggacagctgtggggactgattgcctgccaccatcagacaccctacgtgctgccacccgatctgaggaccacactggagtatctggggcgcctgctgtctctgcaggtccaggtgaaagaagcagccgacgtcgctgcattccgacagagtctgcgagagcaccatgcacgggtggccctggccgctgcacactcactgagccctcatgacacactgagcgatccagctctggacctgctgggactgatgagagcaggaggactgatcctgagatttgaaggcaggtggcagactctgggagaggtccctccagcaccagctgtggacgctctgctggcatggctggagacccagccaggagctctggtgcagacagatgcactgggacagctgtggccagcaggagcagacctggctccttcagcagctggactgctggccatttccgtcggagaaggatggtctgagtgtctggtgtggctgcgcccagaactgcgactggaggtggcttggggaggagcaacccctgatcaggcaaaggacgatctgggaccacgccacagctttgacacatacctggaggaaaaacgaggctatgccgagccctggcacccaggggaaattgaggaggcacaggatctgagagacacactgacaggggcactgggggagagactgtccgtgattcgcgatctcaaccgggctctgacccagtccaatgccgagtggcgtcagtatggcttcgtcatcagtcaccacatgcaggaacccgtcagactgatctcccagtttgccgagcttctgactcgccaacccagagcccaggatggcagcccggactctccccagacagagcgtatcaccggctttctgctcagggaaacctcacgactccgctctctgacccaggacttgcacacgtacactgcgctgctgtcagcacctcctccagttaggaggccaacaccacttgggcgagttgtggacgatgtgctgcaggacctcgaaccacggattgccgatacaggggcctccatagaggtagctcccgaactgcccgtcattgccgctgatgctggcctcttgcgcgaccttctgctgcatctgattggtaacgccttgaccttcggaggaccagagcctcggattgctgtgagaaccgaacggcaaggtgccggctggagcatcgctgtgagcgatcagggtgcggggatagcgccggagtatcaggagaggatcttcttgctcttccagagactcggctctctggacgaggcactgggcaatggacttgggcttcccctgtgtcggaagatcgccgaactgcatggtggcacactgactgtggagagtgcacctggcgaaggaagcacgtttaggtgctggctgcctgatgccggaccactgcctggagcagcagacgcttaa

SEQ ID NO: 13 - DNA, 3201 bp, synthetic construct
  misc_feature 1..3201: note = NLS-DrBphP-CreC60
  source 1..3201: mol_type = other DNA
atggtgcccaagaagaagaggaaagtcggcggaatgagccgcgaccccctgccattcttcccccccctgtacctgggaggacccgagattaccaccgaaaactgtgaacgagagcctatccacatccccggaagtattcagcctcatggcgccctgctgactgctgatggccacagtggggaagtgctgcagatgtcactgaacgccgctaccttcctggggcaggagcctactgtgctgaggggacagaccctggcagcactgctgcctgaacagtggccagcactgcaggctgcactgccacctggctgccccgatgccctgcagtacagggctactctggactggcctgcagctggacacctgagcctgaccgtccatcgcgtgggggaactgctgatcctggagttcgaaccaacagaggcttgggatagcactggcccccacgcactgcggaacgctatgtttgcactggagtccgcccccaatctgagagcactggccgaagtcgccactcagaccgtgcgggagctgacagggttcgatagagtcatgctgtacaagtttgcccctgacgctactggagaagtgatcgctgaagcacggagagaggggctgcacgctttcctgggacatcgatttccagcctccgacattccagcacaggctcgggcactgtataccaggcacctgctgcgactgacagcagatactcgcgcagcagctgtcccactggaccccgtgctgaaccctcagaccaatgcaccaacacctctgggaggagcagtgctgagagcaacctctccaatgcatatgcagtatctgaggaatatgggagtcggcagctccctgtctgtgagtgtggtcgtgggaggacagctgtggggactgattgcctgccaccatcagacaccctacgtgctgccacccgatctgaggaccacactggagtatctggggcgcctgctgtctctgcaggtccaggtgaaagaagcagccgacgtcgctgcattccgacagagtctgcgagagcaccatgcacgggtggccctggccgctgcacactcactgagccctcatgacacactgagcgatccagctctggacctgctgggactgatgagagcaggaggactgatcctgagatttgaaggcaggtggcagactctgggagaggtccctccagcaccagctgtggacgctctgctggcatggctggagacccagccaggagctctggtgcagacagatgcactgggacagctgtggccagcaggagcagacctggctccttcagcagctggactgctggccatttccgtcggagaaggatggtctgagtgtctggtgtggctgcgcccagaactgcgactggaggtggcttggggaggagcaacccctgatcaggcaaaggacgatctgggaccacgccacagctttgacacatacctggaggaaaaacgaggctatgccgagccctggcacccaggggaaattgaggaggcacaggatctgagagacacactgacaggggcactgggggagagactgtccgtgattcgcgatctcaaccgggctctgacccagtccaatgccgagtggcgtcagtatggcttcgtcatcagtcaccacatgcaggaacccgtcagactgatctcccagtttgccgagcttctgactcgccaacccagagcccaggatggcagcccggactctccccagacagagcgtatcaccggctttctgctcagggaaacctcacgactccgctctctgacccaggacttgcacacgtacactgcgctgctgtcagcacctcctccagttaggaggccaacaccacttgggcgagttgtggacgatgtgctgcaggacctcgaaccacggattgccgatacaggggcctccatagaggtagctcccgaactgcccgtcattgccgctgatgctggcctcttgcgcgaccttctgctgcatctgattggtaacgccttgaccttcggaggaccagagcctcggattgctgtgagaaccgaacggcaaggtgccggctggagcatcgctgtgagcgatcagggtgcggggatagcgccggagtatcaggagaggatcttcttgctcttccagagactcggctctctggacgaggcactgggcaatggacttgggcttcccctgtgtcggaagatcgccgaactgcatggtggcacactgactgtggagagtgcacctggcgaaggaagcacgtttaggtgctggctgcctgatgccggaccactgcctggagcagcagacgctggtaccgccagcccctctaaccctggagcctccaacggcagcctcgagaacaggaaatggttccctgctgaacctgaggatgtgagggactacctcctgtacctgcaagccagaggcctggctgtgaagaccatccaacagcacctgggccagctcaacatgctgcacaggagatctggcctgcctcgcccttctgactccaatgctgtgtccctggtgatgaggagaatcagaaaggagaatgtggatgctggggagagagccaagcaggccctggcctttgaacgcactgactttgaccaagtcagatccctgatggagaactctgacagatgccaggacatcaggaacctggccttcctgggcattgcctacaacaccctgctgcgcattgccgaaattgccagaatcagagtgaaggacatctcccgcaccgatggtgggagaatgctgatccacattggcaggaccaagaccctggtgtccacagctggtgtggagaaggccctgtccctgggggttaccaagctggtggagagatggatctctgtgtctggtgtggctgatgaccccaacaactacctgttctgccgggtcagaaagaatggtgtggctgccccttctgccacctcccaactgtccacccgggccctggaagggatctttgaggccacccaccgcctgatctatggtgccaaggatgactctgggcagagatacctggcctggtctggccactctgccagagtgggtgctgccagggacatggccagggctggtgtgtccatccctgaaatcatgcaggctggtggctggaccaatgtgaacattgtgatgaactacatcagaaacctggactctgagactggggccatggtgaggctgctcgaagatggggactaa

SEQ ID NO: 14 - DNA, 2472 bp, synthetic construct
  misc_feature 1..2472: note = NLS-DrBphP-CreN59
  source 1..2472: mol_type = other DNA
atggtgcccaagaagaagaggaaagtcggcggaatgagccgcgaccccctgccattcttcccccccctgtacctgggaggacccgagattaccaccgaaaactgtgaacgagagcctatccacatccccggaagtattcagcctcatggcgccctgctgactgctgatggccacagtggggaagtgctgcagatgtcactgaacgccgctaccttcctggggcaggagcctactgtgctgaggggacagaccctggcagcactgctgcctgaacagtggccagcactgcaggctgcactgccacctggctgccccgatgccctgcagtacagggctactctggactggcctgcagctggacacctgagcctgaccgtccatcgcgtgggggaactgctgatcctggagttcgaaccaacagaggcttgggatagcactggcccccacgcactgcggaacgctatgtttgcactggagtccgcccccaatctgagagcactggccgaagtcgccactcagaccgtgcgggagctgacagggttcgatagagtcatgctgtacaagtttgcccctgacgctactggagaagtgatcgctgaagcacggagagaggggctgcacgctttcctgggacatcgatttccagcctccgacattccagcacaggctcgggcactgtataccaggcacctgctgcgactgacagcagatactcgcgcagcagctgtcccactggaccccgtgctgaaccctcagaccaatgcaccaacacctctgggaggagcagtgctgagagcaacctctccaatgcatatgcagtatctgaggaatatgggagtcggcagctccctgtctgtgagtgtggtcgtgggaggacagctgtggggactgattgcctgccaccatcagacaccctacgtgctgccacccgatctgaggaccacactggagtatctggggcgcctgctgtctctgcaggtccaggtgaaagaagcagccgacgtcgctgcattccgacagagtctgcgagagcaccatgcacgggtggccctggccgctgcacactcactgagccctcatgacacactgagcgatccagctctggacctgctgggactgatgagagcaggaggactgatcctgagatttgaaggcaggtggcagactctgggagaggtccctccagcaccagctgtggacgctctgctggcatggctggagacccagccaggagctctggtgcagacagatgcactgggacagctgtggccagcaggagcagacctggctccttcagcagctggactgctggccatttccgtcggagaaggatggtctgagtgtctggtgtggctgcgcccagaactgcgactggaggtggcttggggaggagcaacccctgatcaggcaaaggacgatctgggaccacgccacagctttgacacatacctggaggaaaaacgaggctatgccgagccctggcacccaggggaaattgaggaggcacaggatctgagagacacactgacaggggcactgggggagagactgtccgtgattcgcgatctcaaccgggctctgacccagtccaatgccgagtggcgtcagtatggcttcgtcatcagtcaccacatgcaggaacccgtcagactgatctcccagtttgccgagcttctgactcgccaacccagagcccaggatggcagcccggactctccccagacagagcgtatcaccggctttctgctcagggaaacctcacgactccgctctctgacccaggacttgcacacgtacactgcgctgctgtcagcacctcctccagttaggaggccaacaccacttgggcgagttgtggacgatgtgctgcaggacctcgaaccacggattgccgatacaggggcctccatagaggtagctcccgaactgcccgtcattgccgctgatgctggcctcttgcgcgaccttctgctgcatctgattggtaacgccttgaccttcggaggaccagagcctcggattgctgtgagaaccgaacggcaaggtgccggctggagcatcgctgtgagcgatcagggtgcggggatagcgccggagtatcaggagaggatcttcttgctcttccagagactcggctctctggacgaggcactgggcaatggacttgggcttcccctgtgtcggaagatcgccgaactgcatggtggcacactgactgtggagagtgcacctggcgaaggaagcacgtttaggtgctggctgcctgatgccggaccactgcctggagcagcagacgctggtaccgccagcccctctaaccctggagcctccaacggcagcctcgagacctctgatgaagtcaggaagaacctgatggacatgttcagggacaggcaggccttctctgaacacacctggaagatgctcctgtctgtgtgcagatcctgggctgcctggtgcaagctgaactaa

SEQ ID NO: 15 - DNA, 2604 bp, synthetic construct
  misc_feature 1..2604: note = NLS-CreN104-DrBphP
  source 1..2604: mol_type = other DNA
atggtgcccaagaagaagaggaaagtcggcggaacctctgatgaagtcaggaagaacctgatggacatgttcagggacaggcaggccttctctgaacacacctggaagatgctcctgtctgtgtgcagatcctgggctgcctggtgcaagctgaacaacaggaaatggttccctgctgaacctgaggatgtgagggactacctcctgtacctgcaagccagaggcctggctgtgaagaccatccaacagcacctgggccagctcaacatgctgcacaggagatctggcctgggtaccgccagcccctctaaccctggagcctccaacggcagcctcgagagccgcgaccccctgccattcttcccccccctgtacctgggaggacccgagattaccaccgaaaactgtgaacgagagcctatccacatccccggaagtattcagcctcatggcgccctgctgactgctgatggccacagtggggaagtgctgcagatgtcactgaacgccgctaccttcctggggcaggagcctactgtgctgaggggacagaccctggcagcactgctgcctgaacagtggccagcactgcaggctgcactgccacctggctgccccgatgccctgcagtacagggctactctggactggcctgcagctggacacctgagcctgaccgtccatcgcgtgggggaactgctgatcctggagttcgaaccaacagaggcttgggatagcactggcccccacgcactgcggaacgctatgtttgcactggagtccgcccccaatctgagagcactggccgaagtcgccactcagaccgtgcgggagctgacagggttcgatagagtcatgctgtacaagtttgcccctgacgctactggagaagtgatcgctgaagcacggagagaggggctgcacgctttcctgggacatcgatttccagcctccgacattccagcacaggctcgggcactgtataccaggcacctgctgcgactgacagcagatactcgcgcagcagctgtcccactggaccccgtgctgaaccctcagaccaatgcaccaacacctctgggaggagcagtgctgagagcaacctctccaatgcatatgcagtatctgaggaatatgggagtcggcagctccctgtctgtgagtgtggtcgtgggaggacagctgtggggactgattgcctgccaccatcagacaccctacgtgctgccacccgatctgaggaccacactggagtatctggggcgcctgctgtctctgcaggtccaggtgaaagaagcagccgacgtcgctgcattccgacagagtctgcgagagcaccatgcacgggtggccctggccgctgcacactcactgagccctcatgacacactgagcgatccagctctggacctgctgggactgatgagagcaggaggactgatcctgagatttgaaggcaggtggcagactctgggagaggtccctccagcaccagctgtggacgctctgctggcatggctggagacccagccaggagctctggtgcagacagatgcactgggacagctgtggccagcaggagcagacctggctccttcagcagctggactgctggccatttccgtcggagaaggatggtctgagtgtctggtgtggctgcgcccagaactgcgactggaggtggcttggggaggagcaacccctgatcaggcaaaggacgatctgggaccacgccacagctttgacacatacctggaggaaaaacgaggctatgccgagccctggcacccaggggaaattgaggaggcacaggatctgagagacacactgacaggggcactgggggagagactgtccgtgattcgcgatctcaaccgggctctgacccagtccaatgccgagtggcgtcagtatggcttcgtcatcagtcaccacatgcaggaacccgtcagactgatctcccagtttgccgagcttctgactcgccaacccagagcccaggatggcagcccggactctccccagacagagcgtatcaccggctttctgctcagggaaacctcacgactccgctctctgacccaggacttgcacacgtacactgcgctgctgtcagcacctcctccagttaggaggccaacaccacttgggcgagttgtggacgatgtgctgcaggacctcgaaccacggattgccgatacaggggcctccatagaggtagctcccgaactgcccgtcattgccgctgatgctggcctcttgcgcgaccttctgctgcatctgattggtaacgccttgaccttcggaggaccagagcctcggattgctgtgagaaccgaacggcaaggtgccggctggagcatcgctgtgagcgatcagggtgcggggatagcgccggagtatcaggagaggatcttcttgctcttccagagactcggctctctggacgaggcactgggcaatggacttgggcttcccctgtgtcggaagatcgccgaactgcatggtggcacactgactgtggagagtgcacctggcgaaggaagcacgtttaggtgctggctgcctgatgccggaccactgcctggagcagcagacgcttaa

SEQ ID NO: 16 - protein, 1016 aa, synthetic construct
  REGION 1..1016: note = NLS-DrBphP-CreC106
VPKKKRKMSRDPLPFFPPLYLGGPEITTENCEREPIHIPGSIQPHGALLTADGHSGEVLQMSLNAATFLGQEPTVLRGQTLAALLPEQWPALQAALPPGCPDALQYRATLDWPAAGHLSLTVHRVGELLILEFEPTEAWDSTGPHALRNAMFALESAPNLRALAEVATQTVRELTGFDRVMLYKFAPDATGEVIAEARREGLHAFLGHRFPASDIPAQARALYTRHLLRLTADTRAAAVPLDPVLNPQTNAPTPLGGAVLRATSPMHMQYLRNMGVGSSLSVSVVVGGQLWGLIACHHQTPYVLPPDLRTTLEYLGRLLSLQVQVKEAADVAAFRQSLREHHARVALAAAHSLSPHDTLSDPALDLLGLMRAGGLILRFEGRWQTLGEVPPAPAVDALLAWLETQPGALVQTDALGQLWPAGADLAPSAAGLLAISVGEGWSECLVWLRPELRLEVAWGGATPDQAKDDLGPRHSFDTYLEEKRGYAEPWHPGEIEEAQDLRDTLTGALGERLSVIRDLNRALTQSNAEWRQYGFVISHHMQEPVRLISQFAELLTRQPRAQDGSPDSPQTERITGFLLRETSRLRSLTQDLHTYTALLSAPPPVRRPTPLGRVVDDVLQDLEPRIADTGASIEVAPELPVIAADAGLLRDLLLHLIGNALTFGGPEPRIAVRTERQGAGWSIAVSDQGAGIAPEYQERIFLLFQRLGSLDEALGNGLGLPLCRKIAELHGGTLTVESAPGEGSTFRCWLPDAGPLPGAADAGTASPSNPGASNGSLERPSDSNAVSLVMRRIRKENVDAGERAKQALAFERTDFDQVRSLMENSDRCQDIRNLAFLGIAYNTLLRIAEIARIRVKDISRTDGGRMLIHIGRTKTLVSTAGVEKALSLGVTKLVERWISVSGVADDPNNYLFCRVRKNGVAAPSATSQLSTRALEGIFEATHRLIYGAKDDSGQRYLAWSGHSARVGAARDMARAGVSIPEIMQAGGWTNVNIVMNYIRNLDSETGAMVRLLEDGD

SEQ ID NO: 17 - DNA, 3063 bp, synthetic construct
  misc_feature 1..3063: note = NLS-DrBphP-CreC106
  source 1..3063: mol_type = other DNA
atggtgcccaagaagaagaggaaagtcggcggaatgagccgcgaccccctgccattcttcccccccctgtacctgggaggacccgagattaccaccgaaaactgtgaacgagagcctatccacatccccggaagtattcagcctcatggcgccctgctgactgctgatggccacagtggggaagtgctgcagatgtcactgaacgccgctaccttcctggggcaggagcctactgtgctgaggggacagaccctggcagcactgctgcctgaacagtggccagcactgcaggctgcactgccacctggctgccccgatgccctgcagtacagggctactctggactggcctgcagctggacacctgagcctgaccgtccatcgcgtgggggaactgctgatcctggagttcgaaccaacagaggcttgggatagcactggcccccacgcactgcggaacgctatgtttgcactggagtccgcccccaatctgagagcactggccgaagtcgccactcagaccgtgcgggagctgacagggttcgatagagtcatgctgtacaagtttgcccctgacgctactggagaagtgatcgctgaagcacggagagaggggctgcacgctttcctgggacatcgatttccagcctccgacattccagcacaggctcgggcactgtataccaggcacctgctgcgactgacagcagatactcgcgcagcagctgtcccactggaccccgtgctgaaccctcagaccaatgcaccaacacctctgggaggagcagtgctgagagcaacctctccaatgcatatgcagtatctgaggaatatgggagtcggcagctccctgtctgtgagtgtggtcgtgggaggacagctgtggggactgattgcctgccaccatcagacaccctacgtgctgccacccgatctgaggaccacactggagtatctggggcgcctgctgtctctgcaggtccaggtgaaagaagcagccgacgtcgctgcattccgacagagtctgcgagagcaccatgcacgggtggccctggccgctgcacactcactgagccctcatgacacactgagcgatccagctctggacctgctgggactgatgagagcaggaggactgatcctgagatttgaaggcaggtggcagactctgggagaggtccctccagcaccagctgtggacgctctgctggcatggctggagacccagccaggagctctggtgcagacagatgcactgggacagctgtggccagcaggagcagacctggctccttcagcagctggactgctggccatttccgtcggagaaggatggtctgagtgtctggtgtggctgcgcccagaactgcgactggaggtggcttggggaggagcaacccctgatcaggcaaaggacgatctgggaccacgccacagctttgacacatacctggaggaaaaacgaggctatgccgagccctggcacccaggggaaattgaggaggcacaggatctgagagacacactgacaggggcactgggggagagactgtccgtgattcgcgatctcaaccgggctctgacccagtccaatgccgagtggcgtcagtatggcttcgtcatcagtcaccacatgcaggaacccgtcagactgatctcccagtttgccgagcttctgactcgccaacccagagcccaggatggcagcccggactctccccagacagagcgtatcaccggctttctgctcagggaaacctcacgactccgctctctgacccaggacttgcacacgtacactgcgctgctgtcagcacctcctccagttaggaggccaacaccacttgggcgagttgtggacgatgtgctgcaggacctcgaaccacggattgccgatacaggggcctccatagaggtagctcccgaactgcccgtcattgccgctgatgctggcctcttgcgcgaccttctgctgcatctgattggtaacgccttgaccttcggaggaccagagcctcggattgctgtgagaaccgaacggcaaggtgccggctggagcatcgctgtgagcgatcagggtgcggggatagcgccggagtatcaggagaggatcttcttgctcttccagagactcggctctctggacgaggcactgggcaatggacttgggcttcccctgtgtcggaagatcgccgaactgcatggtggcacactgactgtggagagtgcacctggcgaaggaagcacgtttaggtgctggctgcctgatgccggaccactgcctggagcagcagacgctggtaccgccagcccctctaaccctggagcctccaacggcagcctcgagcgcccttctgactccaatgctgtgtccctggtgatgaggagaatcagaaaggagaatgtggatgctggggagagagccaagcaggccctggcctttgaacgcactgactttgaccaagtcagatccctgatggagaactctgacagatgccaggacatcaggaacctggccttcctgggcattgcctacaacaccctgctgcgcattgccgaaattgccagaatcagagtgaaggacatctcccgcaccgatggtgggagaatgctgatccacattggcaggaccaagaccctggtgtccacagctggtgtggagaaggccctgtccctgggggttaccaagctggtggagagatggatctctgtgtctggtgtggctgatgaccccaacaactacctgttctgccgggtcagaaagaatggtgtggctgccccttctgccacctcccaactgtccacccgggccctggaagggatctttgaggccacccaccgcctgatctatggtgccaaggatgactctgggcagagatacctggcctggtctggccactctgccagagtgggtgctgccagggacatggccagggctggtgtgtccatccctgaaatcatgcaggctggtggctggaccaatgtgaacattgtgatgaactacatcagaaacctggactctgagactggggccatggtgaggctgctcgaagatggggactaa

SEQ ID NO: 18 - DNA, 2607 bp, synthetic construct
  misc_feature 1..2607: note = NLS-DrBphP-CreN104
  source 1..2607: mol_type = other DNA
atggtgcccaagaagaagaggaaagtcggcggaatgagccgcgaccccctgccattcttcccccccctgtacctgggaggacccgagattaccaccgaaaactgtgaacgagagcctatccacatccccggaagtattcagcctcatggcgccctgctgactgctgatggccacagtggggaagtgctgcagatgtcactgaacgccgctaccttcctggggcaggagcctactgtgctgaggggacagaccctggcagcactgctgcctgaacagtggccagcactgcaggctgcactgccacctggctgccccgatgccctgcagtacagggctactctggactggcctgcagctggacacctgagcctgaccgtccatcgcgtgggggaactgctgatcctggagttcgaaccaacagaggcttgggatagcactggcccccacgcactgcggaacgctatgtttgcactggagtccgcccccaatctgagagcactggccgaagtcgccactcagaccgtgcgggagctgacagggttcgatagagtcatgctgtacaagtttgcccctgacgctactggagaagtgatcgctgaagcacggagagaggggctgcacgctttcctgggacatcgatttccagcctccgacattccagcacaggctcgggcactgtataccaggcacctgctgcgactgacagcagatactcgcgcagcagctgtcccactggaccccgtgctgaaccctcagaccaatgcaccaacacctctgggaggagcagtgctgagagcaacctctccaatgcatatgcagtatctgaggaatatgggagtcggcagctccctgtctgtgagtgtggtcgtgggaggacagctgtggggactgattgcctgccaccatcagacaccctacgtgctgccacccgatctgaggaccacactggagtatctggggcgcctgctgtctctgcaggtccaggtgaaagaagcagccgacgtcgctgcattccgacagagtctgcgagagcaccatgcacgggtggccctggccgctgcacactcactgagccctcatgacacactgagcgatccagctctggacctgctgggactgatgagagcaggaggactgatcctgagatttgaaggcaggtggcagactctgggagaggtccctccagcaccagctgtggacgctctgctggcatggctggagacccagccaggagctctggtgcagacagatgcactgggacagctgtggccagcaggagcagacctggctccttcagcagctggactgctggccatttccgtcggagaaggatggtctgagtgtctggtgtggctgcgcccagaactgcgactggaggtggcttggggaggagcaacccctgatcaggcaaaggacgatctgggaccacgccacagctttgacacatacctggaggaaaaacgaggctatgccgagccctggcacccaggggaaattgaggaggcacaggatctgagagacacactgacaggggcactgggggagagactgtccgtgattcgcgatctcaaccgggctctgacccagtccaatgccgagtggcgtcagtatggcttcgtcatcagtcaccacatgcaggaacccgtcagactgatctcccagtttgccgagcttctgactcgccaacccagagcccaggatggcagcccggactctccccagacagagcgtatcaccggctttctgctcagggaaacctcacgactccgctctctgacccaggacttgcacacgtacactgcgctgctgtcagcacctcctccagttaggaggccaacaccacttgggcgagttgtggacgatgtgctgcaggacctcgaaccacggattgccgatacaggggcctccatagaggtagctcccgaactgcccgtcattgccgctgatgctggcctcttgcgcgaccttctgctgcatctgattggtaacgccttgaccttcggaggaccagagcctcggattgctgtgagaaccgaacggcaaggtgccggctggagcatcgctgtgagcgatcagggtgcggggatagcgccggagtatcaggagaggatcttcttgctcttccagagactcggctctctggacgaggcactgggcaatggacttgggcttcccctgtgtcggaagatcgccgaactgcatggtggcacactgactgtggagagtgcacctggcgaaggaagcacgtttaggtgctggctgcctgatgccggaccactgcctggagcagcagacgctggtaccgccagcccctctaaccctggagcctccaacggcagcctcgagacctctgatgaagtcaggaagaacctgatggacatgttcagggacaggcaggccttctctgaacacacctggaagatgctcctgtctgtgtgcagatcctgggctgcctggtgcaagctgaacaacaggaaatggttccctgctgaacctgaggatgtgagggactacctcctgtacctgcaagccagaggcctggctgtgaagaccatccaacagcacctgggccagctcaacatgctgcacaggagatctggcctgtaa

SEQ ID NO: 19 - DNA, 639 bp, synthetic construct
  misc_feature 1..639: note = Aff6-VP16-NLS
  source 1..639: mol_type = other DNA
atggttgacaacaagtttaacaaggagaagtggcaggctattaaggagattgccgtgctgcctaacctgaaccagccccagcacctggcttttattgtgtctctgctggacgacccttctcagtctgctaacctgctggctgaggctaagaagctgaacgacgctcaggctcctaaggaattcggcggtggaggctcagatagtgctggtagtgctggtagtgctggttccgcgtacagccgcgcgcgtacgaaaaacaattacgggtctaccatcgagggcctgctcgatctcccggacgacgacgcccccgaagaggcggggctggcggctccgcgcctgtcctttctccccgcgggacacacgcgcagactgtcgacggcccccccgaccgatgtcagcctgggggacgagctccacttagacggcgaggacgtggcgatggcgcatgccgacgcgctagacgatttcgatctggacatgttgggggacggggattccccgggtccgggatttaccccccacgactccgccccctacggcgctctggatatggccgacttcgagtttgagcagatgtttaccgatgcccttggaattgacgagtacggtgggcccaagaaaaagcggaaggtgtga

SEQ ID NO: 20 - DNA, 639 bp, synthetic construct
  misc_feature 1..639: note = Aff6_V18F-VP16-NLS
  source 1..639: mol_type = other DNA
atggttgacaacaagtttaacaaggagaagtggcaggctattaaggagattgccttcctgcctaacctgaaccagccccagcacctggcttttattgtgtctctgctggacgacccttctcagtctgctaacctgctggctgaggctaagaagctgaacgacgctcaggctcctaaggaattcggcggtggaggctcagatagtgctggtagtgctggtagtgctggttccgcgtacagccgcgcgcgtacgaaaaacaattacgggtctaccatcgagggcctgctcgatctcccggacgacgacgcccccgaagaggcggggctggcggctccgcgcctgtcctttctccccgcgggacacacgcgcagactgtcgacggcccccccgaccgatgtcagcctgggggacgagctccacttagacggcgaggacgtggcgatggcgcatgccgacgcgctagacgatttcgatctggacatgttgggggacggggattccccgggtccgggatttaccccccacgactccgccccctacggcgctctggatatggccgacttcgagtttgagcagatgtttaccgatgcccttggaattgacgagtacggtgggcccaagaaaaagcggaaggtgtga

SEQ ID NO: 21 - protein, 209 aa, synthetic construct
  REGION 1..209: note = Aff6_V18F N VP16-NLS
MKFNKEKWQAIKEIAFLPNLNQPQHLAFIVSLLDDPSQSANLLAEAKKLNDAQAPKEFGGGGSDSAGSAGSAGSAYSRARTKNNYGSTIEGLLDLPDDDAPEEAGLAAPRLSFLPAGHTRRLSTAPPTDVSLGDELHLDGEDVAMAHADALDDFDLDMLGDGDSPGPGFTPHDSAPYGALDMADFEFEQMFTDALGIDEYGGPKKKRKV

SEQ ID NO: 22 - DNA, 630 bp, synthetic construct
  misc_feature 1..630: note = Aff6_V18F N VP16-NLS
  source 1..630: mol_type = other DNA
atgaagtttaacaaggagaagtggcaggctattaaggagattgccttcctgcctaacctgaaccagccccagcacctggcttttattgtgtctctgctggacgacccttctcagtctgctaacctgctggctgaggctaagaagctgaacgacgctcaggctcctaaggaattcggcggtggaggctcagatagtgctggtagtgctggtagtgctggttccgcgtacagccgcgcgcgtacgaaaaacaattacgggtctaccatcgagggcctgctcgatctcccggacgacgacgcccccgaagaggcggggctggcggctccgcgcctgtcctttctccccgcgggacacacgcgcagactgtcgacggcccccccgaccgatgtcagcctgggggacgagctccacttagacggcgaggacgtggcgatggcgcatgccgacgcgctagacgatttcgatctggacatgttgggggacggggattccccgggtccgggatttaccccccacgactccgccccctacggcgctctggatatggccgacttcgagtttgagcagatgtttaccgatgcccttggaattgacgagtacggtgggcccaagaaaaagcggaaggtgtga

SEQ ID NO: 23 - DNA, 873 bp, synthetic construct
  misc_feature 1..873: note = Aff6_V18F N-3xFLAG-Cfluc
  source 1..873: mol_type = other DNA
atggtgaagtttaacaaggagaagtggcaggctattaaggagattgccttcctgcctaacctgaaccagccccagcacctggcttttattgtgtctctgctggacgacccttctcagtctgctaacctgctggctgaggctaagaagctgaacgacgctcaggctcctaagggcagcgtggactataaggaccacgacggagactacaaggatcatgatattgattacaaagacgatgacgataagggtaccggaggttctggctcaggtagtggaggccccatgatcatgagcggctacgttaacaaccccgaggctacaaacgctctcatcgacaaggacggctggctgcacagcggcgacatcgcctactgggacgaggacgagcacttcttcatcgtggaccggctgaagagcctgatcaaatacaagggctaccaggtagccccagccgaactggagagcatcctgctgcaacaccccaacatcttcgacgccggggtcgccggcctgcccgacgacgatgccggcgagctgcccgccgcagtcgtcgtgctggaacacggtaaaaccatgaccgagaaggagatcgtggactatgtggccagccaggttacaaccgccaagaagctgcgcggtggtgttgtgttcgtggacgaggtgcctaaaggactgaccggcaagttggacgcccgcaagatccgcgagattctcattaaggccaagaagggcggcaagatcgccgtgggatctggaggttcaggaagtggtagtggactcgagtctagagggcccttcgaaggtaagcctatccctaaccctctcctcggtctcgattctacgcgtaccggtcatcatcaccatcaccattga

SEQ ID NO: 24 - DNA, 846 bp, synthetic construct; identical to SEQ ID NO: 8
  misc_feature 1..846: note = 3xNLS-MS2-Aff6_V18F N-V5-His
  source 1..846: mol_type = other DNA

SEQ ID NO: 25 - DNA, 705 bp, synthetic construct
  misc_feature 1..705: note = Aff6_V18F N-MS2-3xNLS
  source 1..705: mol_type = other DNA
atgaagtttaacaaggagaagtggcaggctattaaggagattgccttcctgcctaacctgaaccagccccagcacctggcttttattgtgtctctgctggacgacccttctcagtctgctaacctgctggctgaggctaagaagctgaacgacgctcaggctcctaagggtaccggcggtggaggctcagatagtgctggtagtgccggaagtgcaggcatggcttctaactttactcagttcgttctcgtcgacaatggcggaactggcgacgtgactgtcgccccaagcaacttcgctaacgggatcgctgaatggatcagctctaactcgcgttcacaggcttacaaagtaacctgtagcgttcgtcagagctctgcgcagaatcgcaaatacaccatcaaagtcgaggtgcctaaaggcgcctggcgttcgtacttaaatatggaactaaccattccaattttcgccacgaattccgactgcgagcttattgttaaggcaatgcaaggtctcctaaaagatggaaacccgattccctcagcaatcgcagcaaactccggcatctacgcgctcgagggtggcagcggaggggccagccccaagaagaagcgcaaggtggaagctagcgcttccccgaagaaaaagcggaaagtcgaggcctccgcatctccgaaaaaaaaaagcaaggttgaagcatcttaa

SEQ ID NO: 26 - DNA, 1302 bp, synthetic construct
  misc_feature 1..1302: note = 3xNLS-p65-HSF1-Aff6_V18F N
  source 1..1302: mol_type = other DNA
atggccagccccaagaagaagcgcaaggtggaagctagcgcttccccgaagaaaaagcggaaagtcgaggcctccgcatctccgaaaaaaaaaagcaaggttgaagcatctggatccggtaccggggggagcggcgggccttcagggcagatcagcaaccaggccctggctctggcccctagctccgctccagtgctggcccagactatggtgccctctagtgctatggtgcctctggcccagccacctgctccagcccctgtgctgaccccaggaccaccccagtcactgagcgctccagtgcccaagtctacacaggccggcgaggggactctgagtgaagctctgctgcacctgcagttcgacgctgatgaggacctgggagctctgctggggaacagcaccgatcccggagtgttcacagatctggcctccgtggacaactctgagtttcagcagctgctgaatcagggcgtgtccatgtctcatagtacagccgaaccaatgctgatggagtaccccgaagccattacccggctggtgaccggcagccagcggccccccgaccccgctccaactcccctgggaaccagcggcctgcctaatgggctgtccggagatgaagacttctcaagcatcgctgatatggactttagtgccctgctgtcacagatttcctctagtgggcagggaggaggtggaagcggcttcagcgtggacaccagtgccctgctggacctgttcagcccctcggtgaccgtgcccgacatgagcctgcctgaccttgacagcagcctggccagtatccaagagctcctgtctccccaggagccccccaggcctcccgaggcagagaacagcagcccggattcagggaagcagctggtgcactacacagcgcagccgctgttcctgctggaccccggctccgtggacaccgggagcaacgacctgccggtgctgtttgagctgggagagggctcctacttctccgaaggggacggcttcgccgaggaccccaccatctccctgctgacaggctcggagcctcccaaagccaaggaccccactgtctccctcgagggaggaagtggcagctctggcggcagtggagggtctggtggcagcggaatgaagtttaacaaggagaagtggcaggctattaaggagattgccttcctgcctaacctgaaccagccccagcacctggcttttattgtgtctctgctggacgacccttctcagtctgctaacctgctggctgaggctaagaagctgaacgacgctcaggctcctaagtaa

SEQ ID NO: 27 - DNA, 1290 bp, synthetic construct
  misc_feature 1..1290: note = Aff6_V18F N-p65-HSF1-3xNLS
  source 1..1290: mol_type = other DNA
atgaagtttaacaaggagaagtggcaggctattaaggagattgccttcctgcctaacctgaaccagccccagcacctggcttttattgtgtctctgctggacgacccttctcagtctgctaacctgctggctgaggctaagaagctgaacgacgctcaggctcctaaggaattcggcggtggaggctcagatagtgctggtagtgctggtagtgctggtccttcagggcagatcagcaaccaggccctggctctggcccctagctccgctccagtgctggcccagactatggtgccctctagtgctatggtgcctctggcccagccacctgctccagcccctgtgctgaccccaggaccaccccagtcactgagcgctccagtgcccaagtctacacaggccggcgaggggactctgagtgaagctctgctgcacctgcagttcgacgctgatgaggacctgggagctctgctggggaacagcaccgatcccggagtgttcacagatctggcctccgtggacaactctgagtttcagcagctgctgaatcagggcgtgtccatgtctcatagtacagccgaaccaatgctgatggagtaccccgaagccattacccggctggtgaccggcagccagcggccccccgaccccgctccaactcccctgggaaccagcggcctgcctaatgggctgtccggagatgaagacttctcaagcatcgctgatatggactttagtgccctgctgtcacagatttcctctagtgggcagggaggaggtggaagcggcttcagcgtggacaccagtgccctgctggacctgttcagcccctcggtgaccgtgcccgacatgagcctgcctgaccttgacagcagcctggccagtatccaagagctcctgtctccccaggagccccccaggcctcccgaggcagagaacagcagcccggattcagggaagcagctggtgcactacacagcgcagccgctgttcctgctggaccccggctccgtggacaccgggagcaacgacctgccggtgctgtttgagctgggagagggctcctacttctccgaaggggacggcttcgccgaggaccccaccatctccctgctgacaggctcggagcctcccaaagccaaggaccccactgtctccctcgagggtggcagcggaggggccagccccaagaagaagcgcaaggtggaagctagcgcttccccgaagaaaaagcggaaagtcgaggcctccgcatctccgaaaaaaaaaagcaaggttgaagcatcttaa

SEQ ID NO: 28 - DNA, 924 bp, synthetic construct
  misc_feature 1..924: note = 3xNLS-MS2-2xAff6_V18F N
  source 1..924: mol_type = other DNA
atggccagccccaagaagaagcgcaaggtggaagctagcgcttccccgaagaaaaagcggaaagtcgaggcctccgcatctccaaaaaaaaaaagcaaggttgaagcatctggatccgggggcggaatggcttctaactttactcagttcgttctcgtcgacaatggcggaactggcgacgtgactgtcgccccaagcaacttcgctaacgggatcgctgaatggatcagctctaactcgcgttcacaggcttacaaagtaacctgtagcgttcgtcagagctctgcgcagaatcgcaaatacaccatcaaagtcgaggtgcctaaaggcgcctggcgttcgtacttaaatatggaactaaccattccaattttcgccacgaattccgactgcgagcttattgttaaggcaatgcaaggtctcctaaaagatggaaacccgattccctcagcaatcgcagcaaactccggcatctacgcgggtaccggaggaagtggcagctctggcggcagtggagggtctggtggcagcggaatgaagtttaacaaggagaagtggcaggctattaaggagattgccttcctgcctaacctgaaccagccccagcacctggcttttattgtgtctctgctggacgacccttctcagtctgctaacctgctggctgaggctaagaagctgaacgacgctcaggctcctaaggggggttctggggggagcggcgggggatctggaagtggcagcggaggcctcgagaagtttaacaaggagaagtggcaggctattaaggagattgccttcctgcctaacctgaaccagccccagcacctggcttttattgtgtctctgctggacgacccttctcagtctgctaacctgctggctgaggctaagaagctgaacgacgctcaggctcctaagtaa

SEQ ID NO: 29 - DNA, 906 bp, synthetic construct
  misc_feature 1..906: note = 2xAff6_V18F N-MS2-3xNLS
  source 1..906: mol_type = other DNA
atgaagtttaacaaggagaagtggcaggctattaaggagattgccttcctgcctaacctgaaccagccccagcacctggcttttattgtgtctctgctggacgacccttctcagtctgctaacctgctggctgaggctaagaagctgaacgacgctcaggctcctaagggatccgatagtgctggtagtgccggaagtgcaggcaagtttaacaaggagaagtggcaggctattaaggagattgccttcctgcctaacctgaaccagccccagcacctggcttttattgtgtctctgctggacgacccttctcagtctgctaacctgctggctgaggctaagaagctgaacgacgctcaggctcctaagggtaccggcggtggaggctcagatagtgctggtagtgccggaagtgcaggcatggcttctaactttactcagttcgttctcgtcgacaatggcggaactggcgacgtgactgtcgccccaagcaacttcgctaacgggatcgctgaatggatcagctctaactcgcgttcacaggcttacaaagtaacctgtagcgttcgtcagagctctgcgcagaatcgcaaatacaccatcaaagtcgaggtgcctaaaggcgcctggcgttcgtacttaaatatggaactaaccattccaattttcgccacgaattccgactgcgagcttattgttaaggcaatgcaaggtctcctaaaagatggaaacccgattccctcagcaatcgcagcaaactccggcatctacgcgctcgagggtggcagcggaggggccagccccaagaagaagcgcaaggtggaagctagcgcttccccgaagaaaaagcggaaagtcgaggcctccgcatctccgaaaaaaaaaagcaaggttgaagcatcttaa

SEQ ID NO: 30 - DNA, 372 bp, synthetic construct
  misc_feature 1..372: note = NLS-CreN59-Aff6_V18F N
  source 1..372: mol_type = other DNA
atggtgcccaagaagaagaggaaagtcggcggaacctctgatgaagtcaggaagaacctgatggacatgttcagggacaggcaggccttctctgaacacacctggaagatgctcctgtctgtgtgcagatcctgggctgcctggtgcaagctgaacggtaccgccagcccctctaaccctggagcctccaacggcagcctcgagaagtttaacaaggagaagtggcaggctattaaggagattgccttcctgcctaacctgaaccagccccagcacctggcttttattgtgtctctgctggacgacccttctcagtctgctaacctgctggctgaggctaagaagctgaacgacgctcaggctcctaagtaa

SEQ ID NO: 31 - DNA, 1104 bp, synthetic construct
  misc_feature 1..1104: note = NLS-Aff6_V18F N-CreC60
  source 1..1104: mol_type = other DNA
atggtgcccaagaagaagaggaaagtcggcggaatgaagtttaacaaggagaagtggcaggctattaaggagattgccttcctgcctaacctgaaccagccccagcacctggcttttattgtgtctctgctggacgacccttctcagtctgctaacctgctggctgaggctaagaagctgaacgacgctcaggctcctaagggtaccgccagcccctctaaccctggagcctccaacggcagcctcgagaacaggaaatggttccctgctgaacctgaggatgtgagggactacctcctgtacctgcaagccagaggcctggctgtgaagaccatccaacagcacctgggccagctcaacatgctgcacaggagatctggcctgcctcgcccttctgactccaatgctgtgtccctggtgatgaggagaatcagaaaggagaatgtggatgctggggagagagccaagcaggccctggcctttgaacgcactgactttgaccaagtcagatccctgatggagaactctgacagatgccaggacatcaggaacctggccttcctgggcattgcctacaacaccctgctgcgcattgccgaaattgccagaatcagagtgaaggacatctcccgcaccgatggtgggagaatgctgatccacattggcaggaccaagaccctggtgtccacagctggtgtggagaaggccctgtccctgggggttaccaagctggtggagagatggatctctgtgtctggtgtggctgatgaccccaacaactacctgttctgccgggtcagaaagaatggtgtggctgccccttctgccacctcccaactgtccacccgggccctggaagggatctttgaggccacccaccgcctgatctatggtgccaaggatgactctgggcagagatacctggcctggtctggccactctgccagagtgggtgctgccagggacatggccagggctggtgtgtccatccctgaaatcatgcaggctggtggctggaccaatgtgaacattgtgatgaactacatcagaaacctggactctgagactggggccatggtgaggctgctcgaagatggggactaa

SEQ ID NO: 32 - DNA, 375 bp, synthetic construct
  misc_feature 1..375: note = NLS-Aff6_V18F N-CreN59
  source 1..375: mol_type = other DNA
atggtgcccaagaagaagaggaaagtcggcggaatgaagtttaacaaggagaagtggcaggctattaaggagattgccttcctgcctaacctgaaccagccccagcacctggcttttattgtgtctctgctggacgacccttctcagtctgctaacctgctggctgaggctaagaagctgaacgacgctcaggctcctaagggtaccgccagcccctctaaccctggagcctccaacggcagcctcgagacctctgatgaagtcaggaagaacctgatggacatgttcagggacaggcaggccttctctgaacacacctggaagatgctcctgtctgtgtgcagatcctgggctgcctggtgcaagctgaactaa

SEQ ID NO: 33 - protein, 157 aa, synthetic construct
  REGION 1..157: note = NLS-CreN104-Aff6_V18F N
VPKKKRKVGGTSDEVRKNLMDMFRDRQAFSEHTWKMLLSVCRSWAAWCKLNNRKWFPAEPEDVRDYLLYLQARGLAVKTIQQHLGQGTASPSNPGASNGSLEKFNKEKWQAIKEIAFLPNLNQPQHLAFIVSLLDDPSQSANLLAEAKKLNDAQAPK

SEQ ID NO: 34 - DNA, 507 bp, synthetic construct
  misc_feature 1..507: note = NLS-CreN104-Aff6_V18F N
  source 1..507: mol_type = other DNA
atggtgcccaagaagaagaggaaagtcggcggaacctctgatgaagtcaggaagaacctgatggacatgttcagggacaggcaggccttctctgaacacacctggaagatgctcctgtctgtgtgcagatcctgggctgcctggtgcaagctgaacaacaggaaatggttccctgctgaacctgaggatgtgagggactacctcctgtacctgcaagccagaggcctggctgtgaagaccatccaacagcacctgggccagctcaacatgctgcacaggagatctggcctgggtaccgccagcccctctaaccctggagcctccaacggcagcctcgagaagtttaacaaggagaagtggcaggctattaaggagattgccttcctgcctaacctgaaccagccccagcacctggcttttattgtgtctctgctggacgacccttctcagtctgctaacctgctggctgaggctaagaagctgaacgacgctcaggctcctaagtaa

SEQ ID NO: 35 - DNA, 966 bp, synthetic construct
  misc_feature 1..966: note = NLS-Aff6_V18F N-CreC106
  source 1..966: mol_type = other DNA
atggtgcccaagaagaagaggaaagtcggcggaatgaagtttaacaaggagaagtggcaggctattaaggagattgccttcctgcctaacctgaaccagccccagcacctggcttttattgtgtctctgctggacgacccttctcagtctgctaacctgctggctgaggctaagaagctgaacgacgctcaggctcctaagggtaccgccagcccctctaaccctggagcctccaacggcagcctcgagcgcccttctgactccaatgctgtgtccctggtgatgaggagaatcagaaaggagaatgtggatgctggggagagagccaagcaggccctggcctttgaacgcactgactttgaccaagtcagatccctgatggagaactctgacagatgccaggacatcaggaacctggccttcctgggcattgcctacaacaccctgctgcgcattgccgaaattgccagaatcagagtgaaggacatctcccgcaccgatggtgggagaatgctgatccacattggcaggaccaagaccctggtgtccacagctggtgtggagaaggccctgtccctgggggttaccaagctggtggagagatggatctctgtgtctggtgtggctgatgaccccaacaactacctgttctgccgggtcagaaagaatggtgtggctgccccttctgccacctcccaactgtccacccgggccctggaagggatctttgaggccacccaccgcctgatctatggtgccaaggatgactctgggcagagatacctggcctggtctggccactctgccagagtgggtgctgccagggacatggccagggctggtgtgtccatccctgaaatcatgcaggctggtggctggaccaatgtgaacattgtgatgaactacatcagaaacctggactctgagactggggccatggtgaggctgctcgaagatggggactaa

SEQ ID NO: 36 - DNA, 510 bp, synthetic construct
  misc_feature 1..510: note = NLS-Aff6_V18F N-CreN104
  source 1..510: mol_type = other DNA
atggtgcccaagaagaagaggaaagtcggcggaatgaagtttaacaaggagaagtggcaggctattaaggagattgccttcctgcctaacctgaaccagccccagcacctggcttttattgtgtctctgctggacgacccttctcagtctgctaacctgctggctgaggctaagaagctgaacgacgctcaggctcctaagggtaccgccagcccctctaaccctggagcctccaacggcagcctcgagacctctgatgaagtcaggaagaacctgatggacatgttcagggacaggcaggccttctctgaacacacctggaagatgctcctgtctgtgtgcagatcctgggctgcctggtgcaagctgaacaacaggaaatggttccctgctgaacctgaggatgtgagggactacctcctgtacctgcaagccagaggcctggctgtgaagaccatccaacagcacctgggccagctcaacatgctgcacaggagatctggcctgtaa

SEQ ID NO: 37 - DNA, 1269 bp, synthetic construct
  misc_feature 1..1269: note = NLS-CreN104-Aff6_V18F N-Venus
  source 1..1269: mol_type = other DNA
atggtgcccaagaagaagaggaaagtcggcggaacctctgatgaagtcaggaagaacctgatggacatgttcagggacaggcaggccttctctgaacacacctggaagatgctcctgtctgtgtgcagatcctgggctgcctggtgcaagctgaacaacaggaaatggttccctgctgaacctgaggatgtgagggactacctcctgtacctgcaagccagaggcctggctgtgaagaccatccaacagcacctgggccagctcaacatgctgcacaggagatctggcctgggtaccgccagcccctctaaccctggagcctccaacggcagcctcgagaagtttaacaaggagaagtggcaggctattaaggagattgccttcctgcctaacctgaaccagccccagcacctggcttttattgtgtctctgctggacgacccttctcagtctgctaacctgctggctgaggctaagaagctgaacgacgctcaggctcctaagggatccgccagcccctctaaccctggagcctccaacggcagcgaattcgtgagcaagggcgaggagctgttcaccggggtggtgcccatcctggtcgagctggacggcgacgtaaacggccacaagttcagcgtgtccggcgagggcgagggcgatgccacctacggcaagctgaccctgaagctgatctgcaccaccggcaagctgcccgtgccctggcccaccctcgtgaccaccctgggctacggcctgcagtgcttcgcccgctaccccgaccacatgaagcagcacgacttcttcaagtccgccatgcccgaaggctacgtccaggagcgcaccatcttcttcaaggacgacggcaactacaagacccgcgccgaggtgaagttcgagggcgacaccctggtgaaccgcatcgagctgaagggcatcgacttcaaggaggacggcaacatcctggggcacaagctggagtacaactacaacagccacaacgtctatatcaccgccgacaagcagaagaacggcatcaaggccaacttcaagatccgccacaacatcgaggacggcggcgtgcagctcgccgaccactaccagcagaacacccccatcggcgacggccccgtgctgctgcccgacaaccactacctgagctaccagtccgccctgagcaaagaccccaacgagaagcgcgatcacatggtcctgctggagttcgtgaccgccgccgggatcactctcggcatggacgagctgtacaagtaa

SEQ ID NO: 38 - DNA, 3630 bp, synthetic construct
  misc_feature 1..3630: note = NLS-CreN104-Aff6_V18F N-P2A-NLS-DrBphP-CreC106
  source 1..3630: mol_type = other DNA
atggtgcccaagaagaagaggaaagtcggcggaacctctgatgaagtcaggaagaacctgatggacatgttcagggacaggcaggccttctctgaacacacctggaagatgctcctgtctgtgtgcagatcctgggctgcctggtgcaagctgaacaacaggaaatggttccctgctgaacctgaggatgtgagggactacctcctgtacctgcaagccagaggcctggctgtgaagaccatccaacagcacctgggccagctcaacatgctgcacaggagatctggcctgggtaccgccagcccctctaaccctggagcctccaacggcagcctcgagaagtttaacaaggagaagtggcaggctattaaggagattgccttcctgcctaacctgaaccagccccagcacctggcttttattgtgtctctgctggacgacccttctcagtctgctaacctgctggctgaggctaagaagctgaacgacgctcaggctcctaagggcagcggcgccaccaacttcagcctgctgaagcaggccggcgacgtggaggagaaccccggccccgtgcccaagaagaagaggaaagtcggcggaatgagccgcgaccccctgccattcttcccccccctgtacctgggaggacccgagattaccaccgaaaactgtgaacgagagcctatccacatccccggaagtattcagcctcatggcgccctgctgactgctgatggccacagtggggaagtgctgcagatgtcactgaacgccgctaccttcctggggcaggagcctactgtgctgaggggacagaccctggcagcactgctgcctgaacagtggccagcactgcaggctgcactgccacctggctgccccgatgccctgcagtacagggctactctggactggcctgcagctggacacctgagcctgaccgtccatcgcgtgggggaactgctgatcctggagttcgaaccaacagaggcttgggatagcactggcccccacgcactgcggaacgctatgtttgcactggagtccgcccccaatctgagagcactggccgaagtcgccactcagaccgtgcgggagctgacagggttcgatagagtcatgctgtacaagtttgcccctgacgctactggagaagtgatcgctgaagcacggagagaggggctgcacgctttcctgggacatcgatttccagcctccgacattccagcacaggctcgggcactgtataccaggcacctgctgcgactgacagcagatactcgcgcagcagctgtcccactggaccccgtgctgaaccctcagaccaatgcaccaacacctctgggaggagcagtgctgagagcaacctctccaatgcatatgcagtatctgaggaatatgggagtcggcagctccctgtctgtgagtgtggtcgtgggaggacagctgtggggactgattgcctgccaccatcagacaccctacgtgctgccacccgatctgaggaccacactggagtatctggggcgcctgctgtctctgcaggtccaggtgaaagaagcagccgacgtcgctgcattccgacagagtctgcgagagcaccatgcacgggtggccctggccgctgcacactcactgagccctcatgacacactgagcgatccagctctggacctgctgggactgatgagagcaggaggactgatcctgagatttgaaggcaggtggcagactctgggagaggtccctccagcaccagctgtggacgctctgctggcatggctggagacccagccaggagctctggtgcagacagatgcactgggacagctgtggccagcaggagcagacctggctccttcagcagctggactgctggccatttccgtcggagaaggatggtctgagtgtctggtgtggctgcgcccagaactgcgactggaggtggcttggggaggagcaacccctgatcaggcaaaggacgatctgggaccacgccacagctttgacacatacctggaggaaaaacgaggctatgccgagccctggcacccaggggaaattgaggaggcacaggatctgagagacacactgacaggggcactgggggagagactgtccgtgattcgcgatctcaaccgggctctgacccagtccaatgccgagtggcgtcagtatggcttcgtcatcagtcaccacatgcaggaacccgtcagactgatctcccagtttgccgagcttctgactcgccaacccagagcccaggatggcagcccggactctccccagacagagcgtatcaccggctttctgctcagggaaacctcacgactccgctctctgacccaggacttgcacacgtacactgcgctgctgtcagcacctcctccagttaggaggccaacaccacttgggcgagttgtggacgatgtgctgcaggacctcgaaccacggattgccgatacaggggcctccatagaggtagctcccgaactgcccgtcattgccgctgatgctggcctcttgcgcgaccttctgctgcatctgattggtaacgccttgaccttcggaggaccagagcctcggattgctgtgagaaccgaacggcaaggtgccggctggagcatcgctgtgagcgatcagggtgcggggatagcgccggagtatcaggagaggatcttcttgctcttccagagactcggctctctggacgaggcactgggcaatggacttgggcttcccctgtgtcggaagatcgccgaactgcatggtggcacactgactgtggagagtgcacctggcgaaggaagcacgtttaggtgctggctgcctgatgccggaccactgcctggagcagcagacgctggtaccgccagcccctctaaccctggagcctccaacggcagcctcgagcgcccttctgactccaatgctgtgtccctggtgatgaggagaatcagaaaggagaatgtggatgctggggagagagccaagcaggccctggcctttgaacgcactgactttgaccaagtcagatccctgatggagaactctgacagatgccaggacatcaggaacctggccttcctgggcattgcctacaacaccctgctgcgcattgccgaaattgccagaatcagagtgaaggacatctcccgcaccgatggtgggagaatgctgatccacattggcaggaccaagaccctggtgtccacagctggtgtggagaaggccctgtccctgggggttaccaagctggtggagagatggatctctgtgtctggtgtggctgatgaccccaacaactacctgttctgccgggtcagaaagaatggtgtggctgccccttctgccacctcccaactgtccacccgggccctggaagggatctttgaggccacccaccgcctgatctatggtgccaaggatgactctgggcagagatacctggcctggtctggccactctgccagagtgggtgctgccagggacatggccagggctggtgtgtccatccctgaaatcatgcaggctggtggctggaccaatgtgaacattgtgatgaactacatcagaaacctggactctgagactggggccatggtgaggctgctcgaagatggggactaa

SEQ ID NO: 39 - DNA, 4160 bp, synthetic construct
  misc_feature 1..4160: note = NLS-CreN104-Aff6_V18F N-IRES-NLS-DrBphP-CreC106
  source 1..4160: mol_type = other DNA
atggtgcccaagaagaagaggaaagtcggcggaacctctgatgaagtcaggaagaacctgatggacatgttcagggacaggcaggccttctctgaacacacctggaagatgctcctgtctgtgtgcagatcctgggctgcctggtgcaagctgaacaacaggaaatggttccctgctgaacctgaggatgtgagggactacctcctgtacctgcaagccagaggcctggctgtgaagaccatccaacagcacctgggccagctcaacatgctgcacaggagatctggcctgggtaccgccagcccctctaaccctggagcctccaacggcagcctcgagaagtttaacaaggagaagtggcaggctattaaggagattgccttcctgcctaacctgaaccagccccagcacctggcttttattgtgtctctgctggacgacccttctcagtctgctaacctgctggctgaggctaagaagctgaacgacgctcaggctcctaagtaacccctctccctcccccccccctaacgttactggccgaagccgcttggaataaggccggtgtgcgtttgtctatatgttattttccaccatattgccgtcttttggcaatgtgagggcccggaaacctggccctgtcttcttgacgagcattcctaggggtctttcccctctcgccaaaggaatgcaaggtctgttgaatgtcgtgaaggaagcagttcctctggaagcttcttgaagacaaacaacgtctgtagcgaccctttgcaggcagcggaaccccccacctggcgacaggtgcctctgcggccaaaagccacgtgtataagatacacctgcaaaggcggcacaaccccagtgccacgttgtgagttggatagttgtggaaagagtcaaatggctctcctcaagcgtattcaacaaggggctgaaggatgcccagaaggtaccccattgtatgggatctgatctggggcctcggtgcacatgctttacatgtgtttagtcgaggttaaaaaaacgtctaggccccccgaaccacggggacgtggttttcctttgaaaaacacgatgataatatggccacagccaccatggtgcccaagaagaagaggaaagtcggcggaatgagccgcgaccccctgccattcttcccccccctgtacctgggaggacccgagattaccaccgaaaactgtgaacgagagcctatccacatccccggaagtattcagcctcatggcgccctgctgactgctgatggccacagtggggaagtgctgcagatgtcactgaacgccgctaccttcctggggcaggagcctactgtgctgaggggacagaccctggcagcactgctgcctgaacagtggccagcactgcaggctgcactgccacctggctgccccgatgccctgcagtacagggctactctggactggcctgcagctggacacctgagcctgaccgtccatcgcgtgggggaactgctgatcctggagttcgaaccaacagaggcttgggatagcactggcccccacgcactgcggaacgctatgtttgcactggagtccgcccccaatctgagagcactggccgaagtcgccactcagaccgtgcgggagctgacagggttcgatagagtcatgctgtacaagtttgcccctgacgctactggagaagtgatcgctgaagcacggagagaggggctgcacgctttcctgggacatcgatttccagcctccgacattccagcacaggctcgggcactgtataccaggcacctgctgcgactgacagcagatactcgcgcagcagctgtcccactggaccccgtgctgaaccctcagaccaatgcaccaacacctctgggaggagcagtgctgagagcaacctctccaatgcatatgcagtatctgaggaatatgggagtcggcagctccctgtctgtgagtgtggtcgtgggaggacagctgtggggactgattgcctgccaccatcagacaccctacgtgctgccacccgatctgaggaccacactggagtatctggggcgcctgctgtctctgcaggtccaggtgaaagaagcagccgacgtcgctgcattccgacagagtctgcgagagcaccatgcacgggtggccctggccgctgcacactcactgagccctcatgacacactgagcgatccagctctggacctgctgggactgatgagagcaggaggactgatcctgagatttgaaggcaggtggcagactctgggagaggtccctccagcaccagctgtggacgctctgctggcatggctggagacccagccaggagctctggtgcagacagatgcactgggacagctgtggccagcaggagcagacctggctccttcagcagctggactgctggccatttccgtcggagaaggatggtctgagtgtctggtgtggctgcgcccagaactgcgactggaggtggcttggggaggagcaacccctgatcaggcaaaggacgatctgggaccacgccacagctttgacacatacctggaggaaaaacgaggctatgccgagccctggcacccaggggaaattgaggaggcacaggatctgagagacacactgacaggggcactgggggagagactgtccgtgattcgcgatctcaaccgggctctgacccagtccaatgccgagtggcgtcagtatggcttcgtcatcagtcaccacatgcaggaacccgtcagactgatctcccagtttgccgagcttctgactcgccaacccagagcccaggatggcagcccggactctccccagacagagcgtatcaccggctttctgctcagggaaacctcacgactccgctctctgacccaggacttgcacacgtacactgcgctgctgtcagcacctcctccagttaggaggccaacaccacttgggcgagttgtggacgatgtgctgcaggacctcgaaccacggattgccgatacaggggcctccatagaggtagctcccgaactgcccgtcattgccgctgatgctggcctcttgcgcgaccttctgctgcatctgattggtaacgccttgaccttcggaggaccagagcctcggattgctgtgagaaccgaacggcaaggtgccggctggagcatcgctgtgagcgatcagggtgcggggatagcgccggagtatcaggagaggatcttcttgctcttccagagactcggctctctggacgaggcactgggcaatggacttgggcttcccctgtgtcggaagatcgccgaactgcatggtggcacactgactgtggagagtgcacctggcgaaggaagcacgtttaggtgctggctgcctgatgccggaccactgcctggagcagcagacgctggtaccgccagcccctctaaccctggagcctccaacggcagcctcgagcgcccttctgactccaatgctgtgtccctggtgatgaggagaatcagaaaggagaatgtggatgctggggagagagccaagcaggccctggcctttgaacgcactgactttgaccaagtcagatccctgatggagaactctgacagatgccaggacatcaggaacctggccttcctgggcattgcctacaacaccctgctgcgcattgccgaaattgccagaatcagagtgaaggacatctcccgcaccgatggtgggagaatgctgatccacattggcaggaccaagaccctggtgtccacagctggtgtggagaaggccctgtccctgggggttaccaagctggtggagagatggatctctgtgtctggtgtggctgatgaccccaacaactacctgttctgccgggtcagaaagaatggtgtggctgccccttctgccacctcccaactgtccacccgggccctggaagggatctttgaggccacccaccgcctgatctatggtgccaaggatgactctgggcagagatacctggcctggtctggccactctgccagagtgggtgctgccagggacatggccagggctggtgtgtccatccctgaaatcatgcaggctggtggctggaccaatgtgaacattgtgatgaactacatcagaaacctggactctgagactggggccatggtgaggctgctcgaagatggggactaa

SEQ ID NO: 40 - DNA, 4160 bp, synthetic construct
  misc_feature 1..4160: note = NLS-DrBphP-CreC106-IRES-NLS-CreN104-Aff6_V18F N
  source 1..4160: mol_type = other DNA
atggtgcccaagaagaagaggaaagtcggcggaatgagccgcgaccccctgccattcttcccccccctgtacctgggaggacccgagattaccaccgaaaactgtgaacgagagcctatccacatccccggaagtattcagcctcatggcgccctgctgactgctgatggccacagtggggaagtgctgcagatgtcactgaacgccgctaccttcctggggcaggagcctactgtgctgaggggacagaccctggcagcactgctgcctgaacagtggccagcactgcaggctgcactgccacctggctgccccgatgccctgcagtacagggctactctggactggcctgcagctggacacctgagcctgaccgtccatcgcgtgggggaactgctgatcctggagttcgaaccaacagaggcttgggatagcactggcccccacgcactgcggaacgctatgtttgcactggagtccgcccccaatctgagagcactggccgaagtcgccactcagaccgtgcgggagctgacagggttcgatagagtcatgctgtacaagtttgcccctgacgctactggagaagtgatcgctgaagcacggagagaggggctgcacgctttcctgggacatcgatttccagcctccgacattccagcacaggctcgggcactgtataccaggcacctgctgcgactgacagcagatactcgcgcagcagctgtcccactggaccccgtgctgaaccctcagaccaatgcaccaacacctctgggaggagcagtgctgagagcaacctctccaatgcatatgcagtatctgaggaatatgggagtcggcagctccctgtctgtgagtgtggtcgtgggaggacagctgtggggactgattgcctgccaccatcagacaccctacgtgctgccacccgatctgaggaccacactggagtatctggggcgcctgctgtctctgcaggtccaggtgaaagaagcagccgacgtcgctgcattccgacagagtctgcgagagcaccatgcacgggtggccctggccgctgcacactcactgagccctcatgacacactgagcgatccagctctggacctgctgggactgatgagagcaggaggactgatcctgagatttgaaggcaggtggcagactctgggagaggtccctccagcaccagctgtggacgctctgctggcatggctggagacccagccaggagctctggtgcagacagatgcactgggacagctgtggccagcaggagcagacctggctccttcagcagctggactgctggccatttccgtcggagaaggatggtctgagtgtctggtgtggctgcgcccagaactgcgactggaggtggcttggggaggagcaacccctgatcaggcaaaggacgatctgggaccacgccacagctttgacacatacctggaggaaaaacgaggctatgccgagccctggcacccaggggaaattgaggaggcacaggatctgagagacacactgacaggggcactgggggagagactgtccgtgattcgcgatctcaaccgggctctgacccagtccaatgccgagtggcgtcagtatggcttcgtcatcagtcaccacatgcaggaacccgtcagactgatctcccagtttgccgagcttctgactcgccaacccagagcccaggatggcagcccggactctccccagacagagcgtatcaccggctttctgctcagggaaacctcacgactccgctctctgacccaggacttgcacacgtacactgcgctgctgtcagcacctcctccagttaggaggccaacaccacttgggcgagttgtggacgatgtgctgcaggacctcgaaccacggattgccgatacaggggcctccatagaggtagctcccgaactgcccgtcattgccgctgatgctggcctcttgcgcgaccttctgctgcatctgattggtaacgccttgaccttcggaggaccagagcctcggattgctgtgagaaccgaacggcaaggtgccggctggagcatcgctgtgagcgatcagggtgcggggatagcgccggagtatcaggagaggatcttcttgctcttccagagactcggctctctggacgaggcactgggcaatggacttgggcttcccctgtgtcggaagatcgccgaactgcatggtggcacactgactgtggagagtgcacctggcgaaggaagcacgtttaggtgctggctgcctgatgccggaccactgcctggagcagcagacgctggtaccgccagcccctctaaccctggagcctccaacggcagcctcgagcgcccttctgactccaatgctgtgtccctggtgatgaggagaatcagaaaggagaatgtggatgctggggagagagccaagcaggccctggcctttgaacgcactgactttgaccaagtcagatccctgatggagaactctgacagatgccaggacatcaggaacctggccttcctgggcattgcctacaacaccctgctgcgcattgccgaaattgccagaatcagagtgaaggacatctcccgcaccgatggtgggagaatgctgatccacattggcaggaccaagaccctggtgtccacagctggtgtggagaaggccctgtccctgggggttaccaagctggtggagagatggatctctgtgtctggtgtggctgatgaccccaacaactacctgttctgccgggtcagaaagaatggtgtggctgccccttctgccacctcccaactgtccacccgggccctggaagggatctttgaggccacccaccgcctgatctatggtgccaaggatgactctgggcagagatacctggcctggtctggccactctgccagagtgggtgctgccagggacatggccagggctggtgtgtccatccctgaaatcatgcaggctggtggctggaccaatgtgaacattgtgatgaactacatcagaaacctggactctgagactggggccatggtgaggctgctcgaagatggggactaacccctctccctcccccccccctaacgttactggccgaagccgcttggaataaggccggtgtgcgtttgtctatatgttattttccaccatattgccgtcttttggcaatgtgagggcccggaaacctggccctgtcttcttgacgagcattcctaggggtctttcccctctcgccaaaggaatgcaaggtctgttgaatgtcgtgaaggaagcagttcctctggaagcttcttgaagacaaacaacgtctgtagcgaccctttgcaggcagcggaaccccccacctggcgacaggtgcctctgcggccaaaagccacgtgtataagatacacctgcaaaggcggcacaaccccagtgccacgttgtgagttggatagttgtggaaagagtcaaatggctctcctcaagcgtattcaacaaggggctgaaggatgcccagaaggtaccccattgtatgggatctgatctggggcctcggtgcacatgctttacatgtgtttagtcgaggttaaaaaaacgtctaggccccccgaaccacggggacgtggttttcctttgaaaaacacgatgataatatggccacagccaccatggtgcccaagaagaagaggaaagtcggcggaacctctgatgaagtcaggaagaacctgatggacatgttcagggacaggcaggccttctctgaacacacctggaagatgctcctgtctgtgtgcagatcctgggctgcctggtgcaagctgaacaacaggaaatggttccctgctgaacctgaggatgtgagggactacctcctgtacctgcaagccagaggcctggctgtgaagaccatccaacagcacctgggccagctcaacatgctgcacaggagatctggcctgggtaccgccagcccctctaaccctggagcctccaacggcagcctcgagaagtttaacaaggagaagtggcaggctattaaggagattgccttcctgcctaacctgaaccagccccagcacctggcttttattgtgtctctgctggacgacccttctcagtctgctaacctgctggctgaggctaagaagctgaacgacgctcaggctcctaagtaa

SEQ ID NO: 41 - protein, 58 aa, synthetic construct
  REGION 1..58: note = binder candidate No.1
VDNKFNKEVWSATSEILWLPNLNQLQYFAFIDSLLDDPSQSANLLAEAKKLNDAQAPK

SEQ ID NO: 42 - protein, 58 aa, synthetic construct
  REGION 1..58: note = binder candidate No.2
VDNKFNKELFAAWREIDTLPNLNPSQIWAFIRSLVDDPSQSANLLAEAKKLNDAQAPK

SEQ ID NO: 43 - protein, 58 aa, synthetic construct
  REGION 1..58: note = binder candidate No.3
VDNKFNKEYVRARFEIPLLPNLNPGQWDAFIPSLIDDPSQSANLLAEAKKLNDAQAPK

SEQ ID NO: 44 - protein, 58 aa, synthetic construct
  REGION 1..58: note = binder candidate No.4
VDNKFNKEYVRARFEIPLLPNLNSGQWDAFIPSLIDDPSQSANLLAEAKKLNDAQAPK

SEQ ID NO: 45 - protein, 58 aa, synthetic construct
  REGION 1..58: note = binder candidate No.5
VDNKFNKESLIAQLEIAWLPNLNTSQVVAFIWSLADDPSQSANLLAEAKKLNDAQAPK

SEQ ID NO: 46 - protein, 58 aa, synthetic construct; identical to SEQ ID NO: 1
  REGION 1..58: note = binder candidate No.6

SEQ ID NO: 47 - protein, 58 aa, synthetic construct
  REGION 1..58: note = binder candidate No.7
VDNKFNKEYRVAFLEISWLPNLNVIQATAFIKSLADDPSQSANLLAEAKKLNDAQAPK

SEQ ID NO: 48 - protein, 58 aa, synthetic construct
  REGION 1..58: note = binder candidate No.8
VDNKFNKERFFALSEILWLPNLNWEQLTAFIQSLFDDPSQSANLLAEAKKLNDAQAPK

SEQ ID NO: 49 - protein, 58 aa, synthetic construct
  REGION 1..58: note = binder candidate No.9
VDNKFNKEWWLAIAEIIMLPNLNMTQWPAFIWSLQDDPSQSANLLAEAKKLNDAQAPK

SEQ ID NO: 50 - protein, 58 aa, synthetic construct
  REGION 1..58: note = binder candidate No.10
VDNKFNKEPFCAWLEIQILPNLNTLQIAAFIPSLVDDPSQSANLLAEAKKLNDAQAPK

SEQ ID NO: 51 - protein, 1399 aa, synthetic construct
  REGION 1..1399: note = NLS-dCas9-NLS
MYPYDVPDYASPKKKRKVEASDKKYSIGLAIGTNSVGWAVITDEYKVPSKKFKVLGNTDRHSIKKNLIGALLFDSGETAEATRLKRTARRRYTRRKNRICYLQEIFSNEMAKVDDSFFHRLEESFLVEEDKKHERHPIFGNIVDEVAYHEKYPTIYHLRKKLVDSTDKADLRLIYLALAHMIKFRGHFLIEGDLNPDNSDVDKLFIQLVQTYNQLFEENPINASGVDAKAILSARLSKSRRLENLIAQLPGEKKNGLFGNLIALSLGLTPNFKSNFDLAEDAKLQLSKDTYDDDLDNLLAQIGDQYADLFLAAKNLSDAILLSDILRVNTEITKAPLSASMIKRYDEHHQDLTLLKALVRQQLPEKYKEIFFDQSKNGYAGYIDGGASQEEFYKFIKPILEKMDGTEELLVKLNREDLLRKQRTFDNGSIPHQIHLGELHAILRRQEDFYPFLKDNREKIEKILTFRIPYYVGPLARGNSRFAWMTRKSEETITPWNFEEVVDKGASAQSFIERMTNFDKNLPNEKVLPKHSLLYEYFTVYNELTKVKYVTEGMRKPAFLSGEQKKAIVDLLFKTNRKVTVKQLKEDYFKKIECFDSVEISGVEDRFNASLGTYHDLLKIIKDKDFLDNEENEDILEDIVLTLTLFEDREMIEERLKTYAHLFDDKVMKQLKRRRYTGWGRLSRKLINGIRDKQSGKTILDFLKSDGFANRNFMQLIHDDSLTFKEDIQKAQVSGQGDSLHEHIANLAGSPAIKKGILQTVKVVDELVKVMGRHKPENIVIEMARENQTTQKGQKNSRERMKRIEEGIKELGSQILKEHPVENTQLQNEKLYLYYLQNGRDMYVDQELDINRLSDYDVDAIVPQSFLKDDSIDNKVLTRSDKNRGKSDNVPSEEVVKKMKNYWRQLLNAKLITQRKFDNLTKAERGGLSELDKAGFIKRQLVETRQITKHVAQILDSRMNTKYDENDKLIREVKVITLKSKLVSDFRKDFQFYKVREINNYHHAHDAYLNAVVGTALIKKYPKLESEFVYGDYKVYDVRKMIAKSEQEIGKATAKYFFYSNIMNFFKTEITLANGEIRKRPLIETNGETGEIVWDKGRDFATVRKVLSMPQVNIVKKTEVQTGGFSKESILPKRNSDKLIARKKDWDPKKYGGFDSPTVAYSVLVVAKVEKGKSKKLKSVKELLGITIMERSSFEKNPIDFLEAKGYKEVKKDLIIKLPKYSLFELENGRKRMLASAGELQKGNELALPSKYVNFLYLASHYEKLKGSPEDNEQKQLFVEQHKHYLDEIIEQISEFSKRVILADANLDKVLSAYNKHRDKPIREQAENIIHLFTLTNLGAPAAFKYFDTTIDRKRYTSTKEVLDATLIHQSITGLYETRIDLSQLGGDSPKKKRKVEAS

SEQ ID NO: 52 - DNA, 4200 bp, synthetic construct
  misc_feature 1..4200: note = NLS-dCas9-NLS
  source 1..4200: mol_type = other DNA
atgtacccatacgatgttccagattacgcttcgccgaagaaaaagcgcaaggtcgaagcgtccgacaagaagtacagcatcggcctggccatcggcaccaactctgtgggctgggccgtgatcaccgacgagtacaaggtgcccagcaagaaattcaaggtgctgggcaacaccgaccggcacagcatcaagaagaacctgatcggagccctgctgttcgacagcggcgaaacagccgaggccacccggctgaagagaaccgccagaagaagatacaccagacggaagaaccggatctgctatctgcaagagatcttcagcaacgagatggccaaggtggacgacagcttcttccacagactggaagagtccttcctggtggaagaggataagaagcacgagcggcaccccatcttcggcaacatcgtggacgaggtggcctaccacgagaagtaccccaccatctaccacctgagaaagaaactggtggacagcaccgacaaggccgacctgcggctgatctatctggccctggcccacatgatcaagttccggggccacttcctgatcgagggcgacctgaaccccgacaacagcgacgtggacaagctgttcatccagctggtgcagacctacaaccagctgttcgaggaaaaccccatcaacgccagcggcgtggacgccaaggccatcctgtctgccagactgagcaagagcagacggctggaaaatctgatcgcccagctgcccggcgagaagaagaatggcctgttcggcaacctgattgccctgagcctgggcctgacccccaacttcaagagcaacttcgacctggccgaggatgccaaactgcagctgagcaaggacacctacgacgacgacctggacaacctgctggcccagatcggcgaccagtacgccgacctgtttctggccgccaagaacctgtccgacgccatcctgctgagcgacatcctgagagtgaacaccgagatcaccaaggcccccctgagcgcctctatgatcaagagatacgacgagcaccaccaggacctgaccctgctgaaagctctcgtgcggcagcagctgcctgagaagtacaaagagattttcttcgaccagagcaagaacggctacgccggctacattgacggcggagccagccaggaagagttctacaagttcatcaagcccatcctggaaaagatggacggcaccgaggaactgctcgtgaagctgaacagagaggacctgctgcggaagcagcggaccttcgacaacggcagcatcccccaccagatccacctgggagagctgcacgccattctgcggcggcaggaagatttttacccattcctgaaggacaaccgggaaaagatcgagaagatcctgaccttccgcatcccctactacgtgggccctctggccaggggaaacagcagattcgcctggatgaccagaaagagcgaggaaaccatcaccccctggaacttcgaggaagtggtggacaagggcgcttccgcccagagcttcatcgagcggatgaccaacttcgataagaacctgcccaacgagaaggtgctgcccaagcacagcctgctgtacgagtacttcaccgtgtataacgagctgaccaaagtgaaatacgtgaccgagggaatgagaaagcccgccttcctgagcggcgagcagaaaaaggccatcgtggacctgctgttcaagaccaaccggaaagtgaccgtgaagcagctgaaagaggactacttcaagaaaatcgagtgcttcgactccgtggaaatctccggcgtggaagatcggttcaacgcctccctgggcacataccacgatctgctgaaaattatcaaggacaaggacttcctggacaatgaggaaaacgaggacattctggaagatatcgtgctgaccctgacactgtttgaggacagagagatgatcgaggaacggctgaaaacctatgcccacctgttcgacgacaaagtgatgaagcagctgaagcggcggagatacaccggctggggcaggctgagccggaagctgatcaacggcatccgggacaagcagtccggcaagacaatcctggatttcctgaagtccgacggcttcgccaacagaaacttcatgcagctgatccacgacgacagcctgacctttaaagaggacatccagaaagcccaggtgtccggccagggcgatagcctgcacgagcacattgccaatctggccggcagccccgccattaagaagggcatcctgcagacagtgaaggtggtggacgagctcgtgaaagtgatgggccggcacaagcccgagaacatcgtgatcgaaatggccagagagaaccagaccacccagaagggacagaagaacagccgcgagagaatgaagcggatcgaagagggcatcaaagagctgggcagccagatcctgaaagaacaccccgtggaaaacacccagctgcagaacgagaagctgtacctgtactacctgcagaatgggcgggatatgtacgtggaccaggaactggacatcaaccggctgtccgactacgatgtggacgccatcgtgcctcagagctttctgaaggacgactccatcgacaacaaggtgctgaccagaagcgacaagaaccggggcaagagcgacaacgtgccctccgaagaggtcgtgaagaagatgaagaactactggcggcagctgctgaacgccaagctgattacccagagaaagttcgacaatctgaccaaggccgagagaggcggcctgagcgaactggataaggccggcttcatcaagagacagctggtggaaacccggcagatcacaaagcacgtggcacagatcctggactcccggatgaacactaagtacgacgagaatgacaagctgatccgggaagtgaaagtgatcaccctgaagtccaagctggtgtccgatttccggaaggatttccagttttacaaagtgcgcgagatcaacaactaccaccacgcccacgacgcctacctgaacgccgtcgtgggaaccgccctgatcaaaaagtaccctaagctggaaagcgagttcgtgtacggcgactacaaggtgtacgacgtgcggaagatgatcgccaagagcgagcaggaaatcggcaaggctaccgccaagtacttcttctacagcaacatcatgaactttttcaagaccgagattaccctggccaacggcgagatccggaagcggcctctgatcgagacaaacggcgaaaccggggagatcgtgtgggataagggccgggattttgccaccgtgcggaaagtgctgagcatgccccaagtgaatatcgtgaaaaagaccgaggtgcagacaggcggcttcagcaaagagtctatcctgcccaagaggaacagcgataagctgatcgccagaaagaaggactgggaccctaagaagtacggcggcttcgacagccccaccgtggcctattctgtgctggtggtggccaaagtggaaaagggcaagtccaagaaactgaagagtgtgaaagagctgctggggatcaccatcatggaaagaagcagcttcgagaagaatcccatcgactttctggaagccaagggctacaaagaagtgaaaaaggacctgatcatcaagctgcctaagtactccctgttcgagctggaaaacggccggaagagaatgctggcctctgccggcgaactgcagaagggaaacgaactggccctgccctccaaatatgtgaacttcctgtacctggccagccactatgagaagctgaagggctcccccgaggataatgagcagaaacagctgtttgtggaacagcacaagcactacctggacgagatcatcgagcagatcagcgagttctccaagagagtgatcctggccgacgctaatctggacaaagtgctgtccgcctacaacaagcaccgggataagcccatcagagagcaggccgagaatatcatccacctgtttaccctgaccaatctgggagcccctgccgccttcaagtactttgacaccaccatcgaccggaagaggtacaccagcaccaaagaggtgctggacgccaccctgatccaccagagcatcaccggcctgtacgagacacggatcgacctgtctcagctgggaggcgacagccccaagaagaagagaaaggtggaggccagctaa

SEQ ID NO: 53 - DNA, 135 bp, synthetic construct
  misc_feature 1..135: note = sgRNA_Gal4UAS
  source 1..135: mol_type = other DNA
gagtactgtcctccgcgaattcgttttagagctaggccaacatgaggatcacccatgtctgcagggcctagcaagttaaaataaggctagtccgttatcaacttgaaaaagtggcaccgagtcggtgcttttttt

SEQ ID NO: 54 - DNA, 133 bp, synthetic construct
  misc_feature 1..133: note = sgRNA_MYOD1
  source 1..133: mol_type = other DNA
gcctgggctccggggcgtttgttttagagctaggccaacatgaggatcacccatgtctgcagggcctagcaagttaaaataaggctagtccgttatcaacttgaaaaagtggcaccgagtcggtgcttttttt

SEQ ID NO: 55 - DNA, 133 bp, synthetic construct
  misc_feature 1..133: note = sgRNA_HBG1
  source 1..133: mol_type = other DNA
ggctagggatgaagaataaagttttagagctaggccaacatgaggatcacccatgtctgcagggcctagcaagttaaaataaggctagtccgttatcaacttgaaaaagtggcaccgagtcggtgcttttttt

SEQ ID NO: 56 - DNA, 134 bp, synthetic construct
  misc_feature 1..134: note = sgRNA_IL1R2
  source 1..134: mol_type = other DNA
gtccttggccacttccccatcgttttagagctaggccaacatgaggatcacccatgtctgcagggcctagcaagttaaaataaggctagtccgttatcaacttgaaaaagtggcaccgagtcggtgcttttttt

SEQ ID NO: 57 - DNA, 133 bp, synthetic construct
  misc_feature 1..133: note = sgRNA_ASCL1
  source 1..133: mol_type = other DNA
gcagccgctcgctgcagcaggttttagagctaggccaacatgaggatcacccatgtctgcagggcctagcaagttaaaataaggctagtccgttatcaacttgaaaaagtggcaccgagtcggtgcttttttt

SEQ ID NO: 58 - DNA, 34 bp, synthetic construct
  misc_feature 1..34: note = MS2 aptamer
  source 1..34: mol_type = other DNA
ggccaacatgaggatcacccatgtctgcagggcc

SEQ ID NO: 59 - protein, 1143 aa, synthetic construct
  REGION 1..1143: note = 3xNLS-DrBphP-p65-HSF1
MASPKKKRKVEASASPKKKRKVEASASPKKKSKVEASGSGTGGSGSSGGSGGSGGSGMSRDPLPFFPPLYLGGPEITTENCEREPIHIPGSIQPHGALLTADGHSGEVLQMSLNAATFLGQEPTVLRGQTLAALLPEQWPALQAALPPGCPDALQYRATLDWPAAGHLSLTVHRVGELLILEFEPTEAWDSTGPHALRNAMFALESAPNLRALAEVATQTVRELTGFDRVMLYKFAPDATGEVIAEARREGLHAFLGHRFPASDIPAQARALYTRHLLRLTADTRAAAVPLDPVLNPQTNAPTPLGGAVLRATSPMHMQYLRNMGVGSSLSVSVVVGGQLWGLIACHHQTPYVLPPDLRTTLEYLGRLLSLQVQVKEAADVAAFRQSLREHHARVALAAAHSLSPHDTLSDPALDLLGLMRAGGLILRFEGRWQTLGEVPPAPAVDALLAWLETQPGALVQTDALGQLWPAGADLAPSAAGLLAISVGEGWSECLVWLRPELRLEVAWGGATPDQAKDDLGPRHSFDTYLEEKRGYAEPWHPGEIEEAQDLRDTLTGALGERLSVIRDLNRALTQSNAEWRQYGFVISHHMQEPVRLISQFAELLTRQPRAQDGSPDSPQTERITGFLLRETSRLRSLTQDLHTYTALLSAPPPVRRPTPLGRVVDDVLQDLEPRIADTGASIEVAPELPVIAADAGLLRDLLLHLIGNALTFGGPEPRIAVRTERQGAGWSIAVSDQGAGIAPEYQERIFLLFQRLGSLDEALGNGLGLPLCRKIAELHGGTLTVESAPGEGSTFRCWLPDAGPLPGAADAGGSGGSGGGSGSGSGGLEPSGQISNQALALAPSSAPVLAQTMVPSSAMVPLAQPPAPAPVLTPGPPQSLSAPVPKSTQAGEGTLSEALLHLQFDADEDLGALLGNSTDPGVFTDLASVDNSEFQQLLNQGVSMSHSTAEPMLMEYPEAITRLVTGSQRPPDPAPTPLGTSGLPNGLSGDEDFSSIADMDFSALLSQISSSGQGGGGSGFSVDTSALLDLFSPSVTVPDMSLPDLDSSLASIQELLSPQEPPRPPEAENSSPDSGKQLVHYTAQPLFLLDPGSVDTGSNDLPVLFELGEGSYFSEGDGFAEDPTISLLTGSEPPKAKDPTVS

SEQ ID NO: 60 - protein, 301 aa, synthetic construct
  REGION 1..301: note = 2xAff6_V18F N-MS2-3xNLS
MKFNKEKWQAIKEIAFLPNLNQPQHLAFIVSLLDDPSQSANLLAEAKKLNDAQAPKGSDSAGSAGSAGKFNKEKWQAIKEIAFLPNLNQPQHLAFIVSLLDDPSQSANLLAEAKKLNDAQAPKGTGGGGSDSAGSAGSAGMASNFTQFVLVDNGGTGDVTVAPSNFANGIAEWISSNSRSQAYKVTCSVRQSSAQNRKYTIKVEVPKGAWRSYLNMELTIPIFATNSDCELIVKAMQGLLKDGNPIPSAIAANSGIYALEGGSGGASPKKKRKVEASASPKKKRKVEASASPKKKSKVEAS

SEQ ID NO: 61 - protein, 58 aa, synthetic construct
  REGION 1..58: note = Aff6_V18F
VDNKFNKEKWQAIKEIAFLPNLNQPQHLAFIVSLLDDPSQSANLLAEAKKLNDAQAPK

SEQ ID NO: 62 - protein, 55 aa, synthetic construct
  REGION 1..55: note = Aff6_V18F N
KFNKEKWQAIKEIAFLPNLNQPQHLAFIVSLLDDPSQSANLLAEAKKLNDAQAPK

SEQ ID NO: 63 - protein, 39 aa, Staphylococcus aureus
  source 1..39: note = Affibody (partial)
VDNKFNKEKWQAIKEIAVLPNLNQPQHLAFIVSLLDDPS

SEQ ID NO: 64 - protein, 39 aa, synthetic construct
  REGION 1..39: note = Aff6_V18F (partial)
VDNKFNKEKWQAIKEIAFLPNLNQPQHLAFIVSLLDDPS

SEQ ID NO: 65 - protein, 36 aa, synthetic construct
  REGION 1..36: note = Aff6_V18F N (partial)
KFNKEKWQAIKEIAFLPNLNQPQHLAFIVSLLDDPS